European Patent Application EP 4 537 839 A2, published April 16, 2025. Title: METHOD AND COMPOSITIONS FOR CELLULAR IMMUNOTHERAPY. Applicant: Fred Hutchinson Cancer Center. Application EP. The sequence listing filed with the application follows.

SEQUENCE LISTING (56 sequences)

SEQ ID NO: 1 - skipped

SEQ ID NO: 2 - DNA, 66 bp, synthetic construct
  misc_feature 1..66: note = Synthetic
  source 1..66: mol_type = other DNA
atgctgctgctggtgaccagcctgctgctgtgcgagctgccccaccccgcctttctgctgatcccc

SEQ ID NO: 3 - DNA, 735 bp, synthetic construct
  misc_feature 1..735: note = Synthetic
  source 1..735: mol_type = other DNA
gacatccagatgacccagaccacctccagcctgagcgccagcctgggcgaccgggtgaccatcagctgccgggccagccaggacatcagcaagtacctgaactggtatcagcagaagcccgacggcaccgtcaagctgctgatctaccacaccagccggctgcacagcggcgtgcccagccggtttagcggcagcggctccggcaccgactacagcctgaccatctccaacctggaacaggaagatatcgccacctacttttgccagcagggcaacacactgccctacacctttggcggcggaacaaagctggaaatcaccggcagcacctccggcagcggcaagcctggcagcggcgagggcagcaccaagggcgaggtgaagctgcaggaaagcggccctggcctggtggcccccagccagagcctgagcgtgacctgcaccgtgagcggcgtgagcctgcccgactacggcgtgagctggatccggcagccccccaggaagggcctggaatggctgggcgtgatctggggcagcgagaccacctactacaacagcgccctgaagagccggctgaccatcatcaaggacaacagcaagagccaggtgttcctgaagatgaacagcctgcagaccgacgacaccgccatctactactgcgccaagcactactactacggcggcagctacgccatggactactggggccagggcaccagcgtgaccgtgagcagc

SEQ ID NO: 4 - DNA, 36 bp, synthetic construct
  misc_feature 1..36: note = Synthetic
  source 1..36: mol_type = other DNA
gaatctaagtacggaccgccctgccccccttgccct

SEQ ID NO: 5 - DNA, 84 bp, synthetic construct
  misc_feature 1..84: note = Synthetic
  source 1..84: mol_type = other DNA
atgttctgggtgctggtggtggtcggaggcgtgctggcctgctacagcctgctggtcaccgtggccttcatcatcttttgggtg

SEQ ID NO: 6 - DNA, 126 bp, synthetic construct
  misc_feature 1..126: note = Synthetic
  source 1..126: mol_type = other DNA
aaacggggcagaaagaaactcctgtatatattcaaacaaccatttatgagaccagtacaaactactcaagaggaagatggctgtagctgccgatttccagaagaagaagaaggaggatgtgaactg

SEQ ID NO: 7 - DNA, 336 bp, synthetic construct
  misc_feature 1..336: note = Synthetic
  source 1..336: mol_type = other DNA
cgggtgaagttcagcagaagcgccgacgcccctgcctaccagcagggccagaatcagctgtacaacgagctgaacctgggcagaagggaagagtacgacgtcctggataagcggagaggccgggaccctgagatgggcggcaagcctcggcggaagaacccccaggaaggcctgtataacgaactgcagaaagacaagatggccgaggcctacagcgagatcggcatgaagggcgagcggaggcggggcaagggccacgacggcctgtatcagggcctgtccaccgccaccaaggatacctacgacgccctgcacatgcaggccctgcccccaagg

SEQ ID NO: 8 - DNA, 72 bp, synthetic construct
  misc_feature 1..72: note = Synthetic
  source 1..72: mol_type = other DNA
ctcgagggcggcggagagggcagaggaagtcttctaacatgcggtgacgtggaggagaatcccggccctagg

SEQ ID NO: 9 - DNA, 1074 bp, synthetic construct
  misc_feature 1..1074: note = Synthetic
  source 1..1074: mol_type = other DNA
atgcttctcctggtgacaagccttctgctctgtgagttaccacacccagcattcctcctgatcccacgcaaagtgtgtaacggaataggtattggtgaatttaaagactcactctccataaatgctacgaatattaaacacttcaaaaactgcacctccatcagtggcgatctccacatcctgccggtggcatttaggggtgactccttcacacatactcctcctctggatccacaggaactggatattctgaaaaccgtaaaggaaatcacagggtttttgctgattcaggcttggcctgaaaacaggacggacctccatgcctttgagaacctagaaatcatacgcggcaggaccaagcaacatggtcagttttctcttgcagtcgtcagcctgaacataacatccttgggattacgctccctcaaggagataagtgatggagatgtgataatttcaggaaacaaaaatttgtgctatgcaaatacaataaactggaaaaaactgtttgggacctccggtcagaaaaccaaaattataagcaacagaggtgaaaacagctgcaaggccacaggccaggtctgccatgccttgtgctcccccgagggctgctggggcccggagcccagggactgcgtctcttgccggaatgtcagccgaggcagggaatgcgtggacaagtgcaaccttctggagggtgagccaagggagtttgtggagaactctgagtgcatacagtgccacccagagtgcctgcctcaggccatgaacatcacctgcacaggacggggaccagacaactgtatccagtgtgcccactacattgacggcccccactgcgtcaagacctgcccggcaggagtcatgggagaaaacaacaccctggtctggaagtacgcagacgccggccatgtgtgccacctgtgccatccaaactgcacctacggatgcactgggccaggtcttgaaggctgtccaacgaatgggcctaagatcccgtccatcgccactgggatggtgggggccctcctcttgctgctggtggtggccctggggatcggcctcttcatgtga

SEQ ID NO: 10 - DNA, 2529 bp, synthetic construct
  misc_feature 1..2529: note = Synthetic
  source 1..2529: mol_type = other DNA
atgctgctgctggtgaccagcctgctgctgtgcgagctgccccaccccgcctttctgctgatccccgacatccagatgacccagaccacctccagcctgagcgccagcctgggcgaccgggtgaccatcagctgccgggccagccaggacatcagcaagtacctgaactggtatcagcagaagcccgacggcaccgtcaagctgctgatctaccacaccagccggctgcacagcggcgtgcccagccggtttagcggcagcggctccggcaccgactacagcctgaccatctccaacctggaacaggaagatatcgccacctacttttgccagcagggcaacacactgccctacacctttggcggcggaacaaagctggaaatcaccggcagcacctccggcagcggcaagcctggcagcggcgagggcagcaccaagggcgaggtgaagctgcaggaaagcggccctggcctggtggcccccagccagagcctgagcgtgacctgcaccgtgagcggcgtgagcctgcccgactacggcgtgagctggatccggcagccccccaggaagggcctggaatggctgggcgtgatctggggcagcgagaccacctactacaacagcgccctgaagagccggctgaccatcatcaaggacaacagcaagagccaggtgttcctgaagatgaacagcctgcagaccgacgacaccgccatctactactgcgccaagcactactactacggcggcagctacgccatggactactggggccagggcaccagcgtgaccgtgagcagcgagagcaagtacggaccgccctgccccccttgccctatgttctgggtgctggtggtggtcggaggcgtgctggcctgctacagcctgctggtcaccgtggccttcatcatcttttgggtgaaacggggcagaaagaaactcctgtatatattcaaacaaccatttatgagaccagtacaaactactcaagaggaagatggctgtagctgccgatttccagaagaagaagaaggaggatgtgaactgcgggtgaagttcagcagaagcgccgacgcccctgcctaccagcagggccagaatcagctgtacaacgagctgaacctgggcagaagggaagagtacgacgtcctggataagcggagaggccgggaccctgagatgggcggcaagcctcggcggaagaacccccaggaaggcctgtataacgaactgcagaaagacaagatggccgaggcctacagcgagatcggcatgaagggcgagcggaggcggggcaagggccacgacggcctgtatcagggcctgtccaccgccaccaaggatacctacgacgccctgcacatgcaggccctgcccccaaggctcgagggcggcggagagggcagaggaagtcttctaacatgcggtgacgtggaggagaatcccggccctaggatgcttctcctggtgacaagccttctgctctgtgagttaccacacccagcattcctcctgatcccacgcaaagtgtgtaacggaataggtattggtgaatttaaagactcactctccataaatgctacgaatattaaacacttcaaaaactgcacctccatcagtggcgatctccacatcctgccggtggcatttaggggtgactccttcacacatactcctcctctggatccacaggaactggatattctgaaaaccgtaaaggaaatcacagggtttttgctgattcaggcttggcctgaaaacaggacggacctccatgcctttgagaacctagaaatcatacgcggcaggaccaagcaacatggtcagttttctcttgcagtcgtcagcctgaacataacatccttgggattacgctccctcaaggagataagtgatggagatgtgataatttcaggaaacaaaaatttgtgctatgcaaatacaataaactggaaaaaactgtttgggacctccggtcagaaaaccaaaattataagcaacagaggtgaaaacagctgcaaggccacaggccaggtctgccatgccttgtgctcccccgagggctgctggggcccggagcccagggactgcgtctcttgccggaatgtcagccgaggcagggaatgcgtggacaagtgcaaccttctggagggtgagccaagggagtttgtggagaactctgagtgcatacagtgccacccagagtgcctgcctcaggccatgaacatcacctgcacaggacggggaccagacaactgtatccagtgtgcccactacattgacggcccccactgcgtcaagacctgcccggcaggagtcatgggagaaaacaacaccctggtctggaagtacgcagacgccggccatgtgtgccacctgtgccatccaaactgcacctacggatgcactgggccaggtcttgaaggctgtccaacgaatgggcctaagatcccgtccatcgccactgggatggtgggggccctcctcttgctgctggtggtggccctggggatcggcctcttcatgtga

SEQ ID NO: 11 - protein, 841 aa, synthetic construct
  REGION 1..841: note = Synthetic
MLLLVTSLLLCELPHPAFLLIPDIQMTQTTSSLSASLGDRVTISCRASQDISKYLNWYQQKPDGTVKLLIYHTSRLHSGVPSRFSGSGSGTDYSLTISNLEQEDIATYFCQQGNTLPYTFGGGTKLEITGSTSGSGKPGSGEGSTKGEVKLQESGPGLVAPSQSLSVTCTVSGVSLPDYGVSWIRQPPRKGLEWLGVIWGSETTYYNSALKSRLTIIKDNSKSQVFLKMNSLQTDDTAIYYCAKHYYYGGSYAMDYWGQGTSVTVSSESKYGPPCPPCPMFWVLVVVGGVLACYSLLVTVAFIIFWVKRGRKKLLYIFKQPFMRPVQTTQEEDGCSCRFEEEEGGCELRVKFSRSADAPAYQQGQNQLYNELNLGRREEYDVLDKRRGRDPEMGGKPRRKNPQEGLYNELQKDKMAEAYSEIGMKGERRRGKGHDGLYQGLSTATKDTYDALHMQALPPRLEGGGEGRGSLLTCGDVEENPGPRMLLLVTSLLLCELPHPAFLLIPRKVCNGIGIGEFKDSLSINATNIKHFKNCTSISGDLHILPVAFRGDSFTHTPPLDPQELDILKTVKEITGFLLIQAWPENRTDLHAFENLEIIRGRTKQHGQFSLAVVSLNITSLGLRSLKEISDGDVIISGNKNLCYANTINWKKLFGTSGQKTKIISNRGENSCKATGQVCHALCSPEGCWGPEPRDCVSCRNVSRGRECVDKCNLLEGEPREFVENSECIQCHPECLPQAMNITCTGRGPDNCIQCAHYIDGPHCVKTCPAGVMGENNTLVWKYADAGHVCHLCHPNCTYGCTGPGLEGCPTNGPKIPSIATGMVGALLLLLVVALGIGLFM

SEQ ID NO: 12 - protein, 15 aa, synthetic construct
  REGION 1..15: note = Synthetic
GGGGSGGGGSGGGGS

SEQ ID NO: 13 - protein, 327 aa, Homo sapiens
ASTKGPSVFPLAPCSRSTSESTAALGCLVKDYFPEPVTVSWNSGALTSGVHTFPAVLQSSGLYSLSSVVTVPSSSLGTKTYTCNVDHKPSNTKVDKRVESKYGPPCPSCPAPEFLGGPSVFLFPPKPKDTLMISRTPEVTCVVVDVSQEDPEVQFNWYVDGVEVHNAKTKPREEQFNSTYRVVSVLTVLHQDWLNGKEYKCKVSNKGLPSSIEKTISKAKGQPREPQVYTLPPSQEEMTKNQVSLTCLVKGFYPSDIAVEWESNGQPENNYKTTPPVLDSDGSFFLYSRLTVDKSRWQEGNVFSCSVMHEALHNHYTQKSLSLSLGK

SEQ ID NO: 14 - protein, 220 aa, Homo sapiens
MLRLLLALNLFPSIQVTGNKILVKQSPMLVAYDNAVNLSCKYSYNLFSREFRASLHKGLDSAVEVCVVYGNYSQQLQVYSKTGFNCDGKLGNESVTFYLQNLYVNQTDIYFCKIEVMYPPPYLDNEKSNGTIIHVKGKHLCPSPLFPGPSKPFWVLVVVGGVLACYSLLVTVAFIIFWVRSKRSRLLHSDYMNMTPRRPGPTRKHYQPYAPPRDFAAYRS

SEQ ID NO: 15 - protein, 255 aa, Homo sapiens
MGNSCYNIVATLLLVLNFERTRSLQDPCSNCPAGTFCDNNRNQICSPCPPNSFSSAGGQRTCDICRQCKGVFRTRKECSSTSNAECDCTPGFHCLGAGCSMCEQDCKQGQELTKKGCKDCCFGTFNDQKRGICRPWTNCSLDGKSVLVNGTKERDVVCGPSPADLSPGASSVTPPAPAREPGHSPQIISFFLALTSTALLFLLFFLTLRFSVVKRGRKKLLYIFKQPFMRPVQTTQEEDGCSCRFPEEEEGGCEL

SEQ ID NO: 16 - protein, 164 aa, Homo sapiens
MKWKALFTAAILQAQLPITEAQSFGLLDPKLCYLLDGILFIYGVILTALFLRVKFSRSADAPAYQQGQNQLYNELNLGRREEYDVLDKRRGRDPEMGGKPQRRKNPQEGLYNELQKDKMAEAYSEIGMKGERRRGKGHDGLYQGLSTATKDTYDALHMQALPPR

SEQ ID NO: 17 - protein, 15 aa, Homo sapiens
EPKSCDKTHTCPPCP

SEQ ID NO: 18 - protein, 12 aa, Homo sapiens
ERKCCVECPPCP

SEQ ID NO: 19 - protein, 61 aa, Homo sapiens
ELKTPLGDTHTCPRCPEPKSCDTPPPCPRCPEPKSCDTPPPCPRCPEPKSCDTPPPCPRCP

SEQ ID NO: 20 - protein, 12 aa, Homo sapiens
ESKYGPPCPSCP

SEQ ID NO: 21 - protein, 12 aa, synthetic construct
  REGION 1..12: note = Synthetic
ESKYGPPCPPCP

SEQ ID NO: 22 - DNA, 26 bp, synthetic construct
  misc_feature 1..26: note = Primer
  source 1..26: mol_type = other DNA
atcaaaagaatagaccgagatagggt

SEQ ID NO: 23 - DNA, 26 bp, synthetic construct
  misc_feature 1..26: note = Primer
  source 1..26: mol_type = other DNA
ccgtacctttaagaccaatgacttac

SEQ ID NO: 24 - DNA, 18 bp, synthetic construct
  misc_feature 1..18: note = Primer
  source 1..18: mol_type = other DNA
ttgagagttttcgccccg

SEQ ID NO: 25 - DNA, 24 bp, synthetic construct
  misc_feature 1..24: note = Primer
  source 1..24: mol_type = other DNA
aatagacagatcgctgagataggt

SEQ ID NO: 26 - DNA, 18 bp, synthetic construct
  misc_feature 1..18: note = Primer
  source 1..18: mol_type = other DNA
caggtatccggtaagcgg

SEQ ID NO: 27 - DNA, 19 bp, synthetic construct
  misc_feature 1..19: note = Primer
  source 1..19: mol_type = other DNA
cgaccagcaaccatagtcc

SEQ ID NO: 28 - DNA, 18 bp, synthetic construct
  misc_feature 1..18: note = Primer
  source 1..18: mol_type = other DNA
tagcggtttgactcacgg

SEQ ID NO: 29 - DNA, 20 bp, synthetic construct
  misc_feature 1..20: note = Primer
  source 1..20: mol_type = other DNA
gcagggagctagaacgattc

SEQ ID NO: 30 - DNA, 22 bp, synthetic construct
  misc_feature 1..22: note = Primer
  source 1..22: mol_type = other DNA
attgtctggtatagtgcagcag

SEQ ID NO: 31 - DNA, 16 bp, synthetic construct
  misc_feature 1..16: note = Primer
  source 1..16: mol_type = other DNA
tcgcaacgggtttgcc

SEQ ID NO: 32 - DNA, 21 bp, synthetic construct
  misc_feature 1..21: note = Primer
  source 1..21: mol_type = other DNA
aggaagatatcgccacctact

SEQ ID NO: 33 - DNA, 20 bp, synthetic construct
  misc_feature 1..20: note = Primer
  source 1..20: mol_type = other DNA
cgggtgaagttcagcagaag

SEQ ID NO: 34 - DNA, 20 bp, synthetic construct
  misc_feature 1..20: note = Primer
  source 1..20: mol_type = other DNA
actgtgtttgctgacgcaac

SEQ ID NO: 35 - DNA, 20 bp, synthetic construct
  misc_feature 1..20: note = Primer
  source 1..20: mol_type = other DNA
atgcttctcctggtgacaag

SEQ ID NO: 36 - protein, 18 aa, synthetic construct
  REGION 1..18: note = Synthetic
GSTSGSGKPGSGEGSTKG

SEQ ID NO: 37 - DNA, 10051 bp, synthetic construct
  misc_feature 1..10051: note = Synthetic
  source 1..10051: mol_type = other DNA
gttagaccagatctgagcctgggagctctctggctaactagggaacccactgcttaagcctcaataaagcttgccttgagtgcttcaagtagtgtgtgcccgtctgttgtgtgactctggtaactagagatccctcagacccttttagtcagtgtggaaaatctctagcagtggcgcccgaacagggacttgaaagcgaaagggaaaccagaggagctctctcgacgcaggactcggcttgctgaagcgcgcacggcaagaggcgaggggcggcgactggtgagtacgccaaaaattttgactagcggaggctagaaggagagagatgggtgcgagagcgtcagtattaagcgggggagaattagatcgatgggaaaaaattcggttaaggccagggggaaagaaaaaatataaattaaaacatatagtatgggcaagcagggagctagaacgattcgcagttaatcctggcctgttagaaacatcagaaggctgtagacaaatactgggacagctacaaccatcccttcagacaggatcagaagaacttagatcattatataatacagtagcaaccctctattgtgtgcatcaaaggatagagataaaagacaccaaggaagctttagacaagatagaggaagagcaaaacaaaagtaagaaaaaagcacagcaagcagcagctgacacaggacacagcaatcaggtcagccaaaattaccctatagtgcagaacatccaggggcaaatggtacatcaggccatatcacctagaactttaaatgcatgggtaaaagtagtagaagagaaggctttcagcccagaagtgatacccatgttttcagcattatcagaaggagccaccccacaagatttaaacaccatgctaaacacagtggggggacatcaagcagccatgcaaatgttaaaagagaccatcaatgaggaagctgcaggcaaagagaagagtggtgcagagagaaaaaagagcagtgggaataggagctttgttccttgggttcttgggagcagcaggaagcactatgggcgcagcgtcaatgacgctgacggtacaggccagacaattattgtctggtatagtgcagcagcagaacaatttgctgagggctattgaggcgcaacagcatctgttgcaactcacagtctggggcatcaagcagctccaggcaagaatcctggctgtggaaagatacctaaaggatcaacagctcctggggatttggggttgctctggaaaactcatttgcaccactgctgtgccttggatctacaaatggcagtattcatccacaattttaaaagaaaaggggggattggggggtacagtgcaggggaaagaatagtagacataatagcaacagacatacaaactaaagaattacaaaaacaaattacaaaaattcaaaattttcgggtttattacagggacagcagagatccagtttggggatcaattgcatgaagaatctgcttagggttaggcgttttgcgctgcttcgcgaggatctgcgatcgctccggtgcccgtcagtgggcagagcgcacatcgcccacagtccccgagaagttggggggaggggtcggcaattgaaccggtgcctagagaaggtggcgcggggtaaactgggaaagtgatgtcgtgtactggctccgcctttttcccgagggtgggggagaaccgtatataagtgcagtagtcgccgtgaacgttctttttcgcaacgggtttgccgccagaacacagctgaagcttcgaggggctcgcatctctccttcacgcgcccgccgccctacctgaggccgccatccacgccggttgagtcgcgttctgccgcctcccgcctgtggtgcctcctgaactgcgtccgccgtctaggtaagtttaaagctcaggtcgagaccgggcctttgtccggcgctcccttggagcctacctagactcagccggctctccacgctttgcctgaccctgcttgctcaactctacgtctttgtttcgttttctgttctgcgccgttacagatccaagctgtgaccggcgcctacggctagcgaattcctcgaggccaccatgctgctgctggtgacaagcctgctgctgtgcgagctgccccaccccgcctttctgctgatcccccaggaacagctcgtcgaaagcggcggcagactggtgacacctggcggcagcctgaccctgagctgcaaggccagcggcttcgacttcagcgcctactacatgagctgggtccgccaggcccctggcaagggactggaatggatcgccaccatctaccccagcagcggcaagacctactacgccacctgggtgaacggacggttcaccatctccagcgacaacgcccagaacaccgtggacctgcagatgaacagcctgacagccgccgaccgggccacctacttttgcgccagagacagctacgccgacgacggcgccctgttcaacatctggggccctggcaccctggtgacaatctctagcggcggaggcggatctggtggcggaggaagtggcggcggaggatctgagctggtgctgacccagagcccctctgtgtctgctgccctgggaagccctgccaagatcacctgtaccctgagcagcgcccacaagaccgacaccatcgactggtatcagcagctgcagggcgaggcccccagatacctgatgcaggtgcagagcgacggcagctacaccaagaggccaggcgtgcccgaccggttcagcggatctagctctggcgccgaccgctacctgatcatccccagcgtgcaggccgatgacgaggccgattactactgtggcgccgactacatcggcggctacgtgttcggcggaggcacccagctgaccgtgaccggcgagtctaagtacggaccgccctgccccccttgccctgcccccgagttcctgggcggacccagcgtgttcctgttcccccccaagcccaaggacaccctgatgatcagccggacccccgaggtgacctgcgtggtggtggacgtgagccaggaagatcccgaggtccagttcaattggtacgtggacggcgtggaagtgcacaacgccaagaccaagcccagagaggaacagttcaacagcacctaccgggtggtgtctgtgctgaccgtgctgcaccaggactggctgaacggcaaagaatacaagtgcaaggtgtccaacaagggcctgcccagcagcatcgaaaagaccatcagcaaggccaagggccagcctcgcgagccccaggtgtacaccctgcctccctcccaggaagagatgaccaagaaccaggtgtccctgacctgcctggtgaagggcttctaccccagcgacatcgccgtggagtgggagagcaacggccagcctgagaacaactacaagaccacccctcccgtgctggacagcgacggcagcttcttcctgtacagccggctgaccgtggacaagagccggtggcaggaaggcaacgtctttagctgcagcgtgatgcacgaggccctgcacaaccactacacccagaagagcctgagcctgtccctgggcaagatgttctgggtgctggtggtggtgggcggggtgctggcctgctacagcctgctggtgacagtggccttcatcatcttttgggtgaaacggggcagaaagaaactcctgtatatattcaaacaaccatttatgagaccagtacaaactactcaagaggaagatggctgtagctgccgatttccagaagaagaagaaggaggatgtgaactgcgggtgaagttcagcagaagcgccgacgcccctgcctaccagcagggccagaatcagctgtacaacgagctgaacctgggcagaagggaagagtacgacgtcctggataagcggagaggccgggaccctgagatgggcggcaagcctcggcggaagaacccccaggaaggcctgtataacgaactgcagaaagacaagatggccgaggcctacagcgagatcggcatgaagggcgagcggaggcggggcaagggccacgacggcctgtatcagggcctgtccaccgccaccaaggatacctacgacgccctgcacatgcaggccctgcccccaaggctcgagggcggcggagagggcagaggaagtcttctaacatgcggtgacgtggaggagaatcccggccctaggatgcttctcctggtgacaagccttctgctctgtgagttaccacacccagcattcctcctgatcccacgcaaagtgtgtaacggaataggtattggtgaatttaaagactcactctccataaatgctacgaatattaaacacttcaaaaactgcacctccatcagtggcgatctccacatcctgccggtggcatttaggggtgactccttcacacatactcctcctctggatccacaggaactggatattctgaaaaccgtaaaggaaatcacagggtttttgctgattcaggcttggcctgaaaacaggacggacctccatgcctttgagaacctagaaatcatacgcggcaggaccaagcaacatggtcagttttctcttgcagtcgtcagcctgaacataacatccttgggattacgctccctcaaggagataagtgatggagatgtgataatttcaggaaacaaaaatttgtgctatgcaaatacaataaactggaaaaaactgtttgggacctccggtcagaaaaccaaaattataagcaacagaggtgaaaacagctgcaaggccacaggccaggtctgccatgccttgtgctcccccgagggctgctggggcccggagcccagggactgcgtctcttgccggaatgtcagccgaggcagggaatgcgtggacaagtgcaaccttctggagggtgagccaagggagtttgtggagaactctgagtgcatacagtgccacccagagtgcctgcctcaggccatgaacatcacctgcacaggacggggaccagacaactgtatccagtgtgcccactacattgacggcccccactgcgtcaagacctgcccggcaggagtcatgggagaaaacaacaccctggtctggaagtacgcagacgccggccatgtgtgccacctgtgccatccaaactgcacctacggatgcactgggccaggtcttgaaggctgtccaacgaatgggcctaagatcccgtccatcgccactgggatggtgggggccctcctcttgctgctggtggtggccctggggatcggcctcttcatgtgagcggccgctctagacccgggctgcaggaattcgatatcaagcttatcgataatcaacctctggattacaaaatttgtgaaagattgactggtattcttaactatgttgctccttttacgctatgtggatacgctgctttaatgcctttgtatcatgctattgcttcccgtatggctttcattttctcctccttgtataaatcctggttgctgtctctttatgaggagttgtggcccgttgtcaggcaacgtggcgtggtgtgcactgtgtttgctgacgcaacccccactggttggggcattgccaccacctgtcagctcctttccgggactttcgctttccccctccctattgccacggcggaactcatcgccgcctgccttgcccgctgctggacaggggctcggctgttgggcactgacaattccgtggtgttgtcggggaaatcatcgtcctttccttggctgctcgcctgtgttgccacctggattctgcgcgggacgtccttctgctacgtcccttcggccctcaatccagcggaccttccttcccgcggcctgctgccggctctgcggcctcttccgcgtcttcgccttcgccctcagacgagtcggatctccctttgggccgcctccccgcatcgataccgtcgactagccgtacctttaagaccaatgacttacaaggcagctgtagatcttagccactttttaaaagaaaaggggggactggaagggctaattcactcccaaagaagacaagatctgctttttgcctgtactgggtctctctggttagaccagatctgagcctgggagctctctggctaactagggaacccactgcttaagcctcaataaagcttgccttgagtgcttcaagtagtgtgtgcccgtctgttgtgtgactctggtaactagagatccctcagacccttttagtcagtgtggaaaatctctagcagaattcgatatcaagcttatcgataccgtcgacctcgagggggggcccggtacccaattcgccctatagtgagtcgtattacaattcactggccgtcgttttacaacgtcgtgactgggaaaaccctggcgttacccaacttaatcgccttgcagcacatccccctttcgccagctggcgtaatagcgaagaggcccgcaccgatcgcccttcccaacagttgcgcagcctgaatggcgaatggaaattgtaagcgttaatattttgttaaaattcgcgttaaatttttgttaaatcagctcattttttaaccaataggccgaaatcggcaaaatcccttataaatcaaaagaatagaccgagatagggttgagtgttgttccagtttggaacaagagtccactattaaagaacgtggactccaacgtcaaagggcgaaaaaccgtctatcagggcgatggcccactacgtgaaccatcaccctaatcaagttttttggggtcgaggtgccgtaaagcactaaatcggaaccctaaagggagcccccgatttagagcttgacggggaaagccggcgaacgtggcgagaaaggaagggaagaaagcgaaaggagcgggcgctagggcgctggcaagtgtagcggtcacgctgcgcgtaaccaccacacccgccgcgcttaatgcgccgctacagggcgcgtcaggtggcacttttcggggaaatgtgcgcggaacccctatttgtttatttttctaaatacattcaaatatgtatccgctcatgagacaataaccctgataaatgcttcaataatattgaaaaaggaagagtatgagtattcaacatttccgtgtcgcccttattcccttttttgcggcattttgccttcctgtttttgctcacccagaaacgctggtgaaagtaaaagatgctgaagatcagttgggtgcacgagtgggttacatcgaactggatctcaacagcggtaagatccttgagagttttcgccccgaagaacgttttccaatgatgagcacttttaaagttctgctatgtggcgcggtattatcccgtattgacgccgggcaagagcaactcggtcgccgcatacactattctcagaatgacttggttgagtactcaccagtcacagaaaagcatcttacggatggcatgacagtaagagaattatgcagtgctgccataaccatgagtgataacactgcggccaacttacttctgacaacgatcggaggaccgaaggagctaaccgcttttttgcacaacatgggggatcatgtaactcgccttgatcgttgggaaccggagctgaatgaagccataccaaacgacgagcgtgacaccacgatgcctgtagcaatggcaacaacgttgcgcaaactattaactggcgaactacttactctagcttcccggcaacaattaatagactggatggaggcggataaagttgcaggaccacttctgcgctcggcccttccggctggctggtttattgctgataaatctggagccggtgagcgtgggtctcgcggtatcattgcagcactggggccagatggtaagccctcccgtatcgtagttatctacacgacggggagtcaggcaactatggatgaacgaaatagacagatcgctgagataggtgcctcactgattaagcattggtaactgtcagaccaagtttactcatatatactttagattgatttaaaacttcatttttaatttaaaaggatctaggtgaagatcctttttgataatctcatgaccaaaatcccttaacgtgagttttcgttccactgagcgtcagaccccgtagaaaagatcaaaggatcttcttgagatcctttttttctgcgcgtaatctgctgcttgcaaacaaaaaaaccaccgctaccagcggtggtttgtttgccggatcaagagctaccaactctttttccgaaggtaactggcttcagcagagcgcagataccaaatactgttcttctagtgtagccgtagttaggccaccacttcaagaactctgtagcaccgcctacatacctcgctctgctaatcctgttaccagtggctgctgccagtggcgataagtcgtgtcttaccgggttggactcaagacgatagttaccggataaggcgcagcggtcgggctgaacggggggttcgtgcacacagcccagcttggagcgaacgacctacaccgaactgagatacctacagcgtgagctatgagaaagcgccacgcttcccgaagggagaaaggcggacaggtatccggtaagcggcagggtcggaacaggagagcgcacgagggagcttccagggggaaacgcctggtatctttatagtcctgtcgggtttcgccacctctgacttgagcgtcgatttttgtgatgctcgtcaggggggcggagcctatggaaaaacgccagcaacgcggcctttttacggttcctggccttttgctggccttttgctcacatgttctttcctgcgttatcccctgattctgtggataaccgtattaccgcctttgagtgagctgataccgctcgccgcagccgaacgaccgagcgcagcgagtcagtgagcgaggaagcggaagagcgcccaatacgcaaaccgcctctccccgcgcgttggccgattcattaatgcagctggcacgacaggtttcccgactggaaagcgggcagtgagcgcaacgcaattaatgtgagttagctcactcattaggcaccccaggctttacactttatgcttccggctcgtatgttgtgtggaattgtgagcggataacaatttcacacaggaaacagctatgaccatgattacgccaagctcgaaattaaccctcactaaagggaacaaaagctggagctccaccgcggtggcggcctcgaggtcgagatccggtcgaccagcaaccatagtcccgcccctaactccgcccatcccgcccctaactccgcccagttccgcccattctccgccccatggctgactaattttttttatttatgcagaggccgaggccgcctcggcctctgagctattccagaagtagtgaggaggcttttttggaggcctaggcttttgcaaaaagcttcgacggtatcgattggctcatgtccaacattaccgccatgttgacattgattattgactagttattaatagtaatcaattacggggtcattagttcatagcccatatatggagttccgcgttacataacttacggtaaatggcccgcctggctgaccgcccaacgacccccgcccattgacgtcaataatgacgtatgttcccatagtaacgccaatagggactttccattgacgtcaatgggtggagtatttacggtaaactgcccacttggcagtacatcaagtgtatcatatgccaagtacgccccctattgacgtcaatgacggtaaatggcccgcctggcattatgcccagtacatgaccttatgggactttcctacttggcagtacatctacgtattagtcatcgctattaccatggtgatgcggttttggcagtacatcaatgggcgtggatagcggtttgactcacggggatttccaagtctccaccccattgacgtcaatgggagtttgttttggcaccaaaatcaacgggactttccaaaatgtcgtaacaactccgccccattgacgcaaatgggcggtaggcgtgtacggaattcggagtggcgagccctcagatcctgcatataagcagctgctttttgcctgtactgggtctctctg

SEQ ID NO: 38 - protein, 1062 aa, synthetic construct
  REGION 1..1062: note = Synthetic
MLLLVTSLLLCELPHPAFLLIPQEQLVESGGRLVTPGGSLTLSCKASGFDFSAYYMSWVRQAPGKGLEWIATIYPSSGKTYYATWVNGRFTISSDNAQNTVDLQMNSLTAADRATYFCARDSYADDGALFNIWGPGTLVTISSGGGGSGGGGSGGGGSELVLTQSPSVSAALGSPAKITCTLSSAHKTDTIDWYQQLQGEAPRYLMQVQSDGSYTKRPGVPDRFSGSSSGADRYLIIPSVQADDEADYYCGADYIGGYVFGGGTQLTVTGESKYGPPCPPCPAPEFLGGPSVFLFPPKPKDTLMISRTPEVTCVVVDVSQEDPEVQFNWYVDGVEVHNAKTKPREEQFNSTYRVVSVLTVLHQDWLNGKEYKCKVSNKGLPSSIEKTISKAKGQPREPQVYTLPPSQEEMTKNQVSLTCLVKGFYPSDIAVEWESNGQPENNYKTTPPVLDSDGSFFLYSRLTVDKSRWQEGNVFSCSVMHEALHNHYTQKSLSLSLGKMFWVLVVVGGVLACYSLLVTVAFIIFWVKRGRKKLLYIFKQPFMRPVQTTQEEDGCSCRFPEEEEGGCELRVKFSRSADAPAYQQGQNQLYNELNLGRREEYDVLDKRRGRDPEMGGKPRRKNPQEGLYNELQKDKMAEAYSEIGMKGERRRGKGHDGLYQGLSTATKDTYDALHMQALPPRLEGGGEGRGSLLTCGDVEENPGPRMLLLVTSLLLCELPHPAFLLIPRKVCNGIGIGEFKDSLSINATNIKHFKNCTSISGDLHILPVAFRGDSFTHTPPLDPQELDILKTVKEITGFLLIQAWPENRTDLHAFENLEIIRGRTKQHGQFSLAVVSLNITSLGLRSLKEISDGDVIISGNKNLCYANTINWKKLFGTSGQKTKIISNRGENSCKATGQVCHALCSPEGCWGPEPRDCVSCRNVSRGRECVDKCNLLEGEPREFVENSECIQCHPECLPQAMNITCTGRGPDNCIQCAHYIDGPHCVKTCPAGVMGENNTLVWKYADAGHVCHLCHPNCTYGCTGPGLEGCPTNGPKIPSIATGMVGALLLLLVVALGIGLFM

SEQ ID NO: 39 - DNA, 9721 bp, synthetic construct
  misc_feature 1..9721: note = Synthetic
  source 1..9721: mol_type = other DNA
gttagaccagatctgagcctgggagctctctggctaactagggaacccactgcttaagcctcaataaagcttgccttgagtgcttcaagtagtgtgtgcccgtctgttgtgtgactctggtaactagagatccctcagacccttttagtcagtgtggaaaatctctagcagtggcgcccgaacagggacttgaaagcgaaagggaaaccagaggagctctctcgacgcaggactcggcttgctgaagcgcgcacggcaagaggcgaggggcggcgactggtgagtacgccaaaaattttgactagcggaggctagaaggagagagatgggtgcgagagcgtcagtattaagcgggggagaattagatcgatgggaaaaaattcggttaaggccagggggaaagaaaaaatataaattaaaacatatagtatgggcaagcagggagctagaacgattcgcagttaatcctggcctgttagaaacatcagaaggctgtagacaaatactgggacagctacaaccatcccttcagacaggatcagaagaacttagatcattatataatacagtagcaaccctctattgtgtgcatcaaaggatagagataaaagacaccaaggaagctttagacaagatagaggaagagcaaaacaaaagtaagaaaaaagcacagcaagcagcagctgacacaggacacagcaatcaggtcagccaaaattaccctatagtgcagaacatccaggggcaaatggtacatcaggccatatcacctagaactttaaatgcatgggtaaaagtagtagaagagaaggctttcagcccagaagtgatacccatgttttcagcattatcagaaggagccaccccacaagatttaaacaccatgctaaacacagtggggggacatcaagcagccatgcaaatgttaaaagagaccatcaatgaggaagctgcaggcaaagagaagagtggtgcagagagaaaaaagagcagtgggaataggagctttgttccttgggttcttgggagcagcaggaagcactatgggcgcagcgtcaatgacgctgacggtacaggccagacaattattgtctggtatagtgcagcagcagaacaatttgctgagggctattgaggcgcaacagcatctgttgcaactcacagtctggggcatcaagcagctccaggcaagaatcctggctgtggaaagatacctaaaggatcaacagctcctggggatttggggttgctctggaaaactcatttgcaccactgctgtgccttggatctacaaatggcagtattcatccacaattttaaaagaaaaggggggattggggggtacagtgcaggggaaagaatagtagacataatagcaacagacatacaaactaaagaattacaaaaacaaattacaaaaattcaaaattttcgggtttattacagggacagcagagatccagtttggggatcaattgcatgaagaatctgcttagggttaggcgttttgcgctgcttcgcgaggatctgcgatcgctccggtgcccgtcagtgggcagagcgcacatcgcccacagtccccgagaagttggggggaggggtcggcaattgaaccggtgcctagagaaggtggcgcggggtaaactgggaaagtgatgtcgtgtactggctccgcctttttcccgagggtgggggagaaccgtatataagtgcagtagtcgccgtgaacgttctttttcgcaacgggtttgccgccagaacacagctgaagcttcgaggggctcgcatctctccttcacgcgcccgccgccctacctgaggccgccatccacgccggttgagtcgcgttctgccgcctcccgcctgtggtgcctcctgaactgcgtccgccgtctaggtaagtttaaagctcaggtcgagaccgggcctttgtccggcgctcccttggagcctacctagactcagccggctctccacgctttgcctgaccctgcttgctcaactctacgtctttgtttcgttttctgttctgcgccgttacagatccaagctgtgaccggcgcctacggctagcgaattcctcgaggccaccatgctgctgctggtgacaagcctgctgctgtgcgagctgccccaccccgcctttctgctgatcccccaggaacagctcgtcgaaagcggcggcagactggtgacacctggcggcagcctgaccctgagctgcaaggccagcggcttcgacttcagcgcctactacatgagctgggtccgccaggcccctggcaagggactggaatggatcgccaccatctaccccagcagcggcaagacctactacgccacctgggtgaacggacggttcaccatctccagcgacaacgcccagaacaccgtggacctgcagatgaacagcctgacagccgccgaccgggccacctacttttgcgccagagacagctacgccgacgacggcgccctgttcaacatctggggccctggcaccctggtgacaatctctagcggcggaggcggatctggtggcggaggaagtggcggcggaggatctgagctggtgctgacccagagcccctctgtgtctgctgccctgggaagccctgccaagatcacctgtaccctgagcagcgcccacaagaccgacaccatcgactggtatcagcagctgcagggcgaggcccccagatacctgatgcaggtgcagagcgacggcagctacaccaagaggccaggcgtgcccgaccggttcagcggatctagctctggcgccgaccgctacctgatcatccccagcgtgcaggccgatgacgaggccgattactactgtggcgccgactacatcggcggctacgtgttcggcggaggcacccagctgaccgtgaccggcgagtctaagtacggaccgccctgccccccttgccctggccagcctcgcgagccccaggtgtacaccctgcctccctcccaggaagagatgaccaagaaccaggtgtccctgacctgcctggtgaagggcttctaccccagcgacatcgccgtggagtgggagagcaacggccagcctgagaacaactacaagaccacccctcccgtgctggacagcgacggcagcttcttcctgtacagccggctgaccgtggacaagagccggtggcaggaaggcaacgtctttagctgcagcgtgatgcacgaggccctgcacaaccactacacccagaagagcctgagcctgtccctgggcaagatgttctgggtgctggtggtggtgggcggggtgctggcctgctacagcctgctggtgacagtggccttcatcatcttttgggtgaaacggggcagaaagaaactcctgtatatattcaaacaaccatttatgagaccagtacaaactactcaagaggaagatggctgtagctgccgatttccagaagaagaagaaggaggatgtgaactgcgggtgaagttcagcagaagcgccgacgcccctgcctaccagcagggccagaatcagctgtacaacgagctgaacctgggcagaagggaagagtacgacgtcctggataagcggagaggccgggaccctgagatgggcggcaagcctcggcggaagaacccccaggaaggcctgtataacgaactgcagaaagacaagatggccgaggcctacagcgagatcggcatgaagggcgagcggaggcggggcaagggccacgacggcctgtatcagggcctgtccaccgccaccaaggatacctacgacgccctgcacatgcaggccctgcccccaaggctcgagggcggcggagagggcagaggaagtcttctaacatgcggtgacgtggaggagaatcccggccctaggatgcttctcctggtgacaagccttctgctctgtgagttaccacacccagcattcctcctgatcccacgcaaagtgtgtaacggaataggtattggtgaatttaaagactcactctccataaatgctacgaatattaaacacttcaaaaactgcacctccatcagtggcgatctccacatcctgccggtggcatttaggggtgactccttcacacatactcctcctctggatccacaggaactggatattctgaaaaccgtaaaggaaatcacagggtttttgctgattcaggcttggcctgaaaacaggacggacctccatgcctttgagaacctagaaatcatacgcggcaggaccaagcaacatggtcagttttctcttgcagtcgtcagcctgaacataacatccttgggattacgctccctcaaggagataagtgatggagatgtgataatttcaggaaacaaaaatttgtgctatgcaaatacaataaactggaaaaaactgtttgggacctccggtcagaaaaccaaaattataagcaacagaggtgaaaacagctgcaaggccacaggccaggtctgccatgccttgtgctcccccgagggctgctggggcccggagcccagggactgcgtctcttgccggaatgtcagccgaggcagggaatgcgtggacaagtgcaaccttctggagggtgagccaagggagtttgtggagaactctgagtgcatacagtgccacccagagtgcctgcctcaggccatgaacatcacctgcacaggacggggaccagacaactgtatccagtgtgcccactacattgacggcccccactgcgtcaagacctgcccggcaggagtcatgggagaaaacaacaccctggtctggaagtacgcagacgccggccatgtgtgccacctgtgccatccaaactgcacctacggatgcactgggccaggtcttgaaggctgtccaacgaatgggcctaagatcccgtccatcgccactgggatggtgggggccctcctcttgctgctggtggtggccctggggatcggcctcttcatgtgagcggccgctctagacccgggctgcaggaattcgatatcaagcttatcgataatcaacctctggattacaaaatttgtgaaagattgactggtattcttaactatgttgctccttttacgctatgtggatacgctgctttaatgcctttgtatcatgctattgcttcccgtatggctttcattttctcctccttgtataaatcctggttgctgtctctttatgaggagttgtggcccgttgtcaggcaacgtggcgtggtgtgcactgtgtttgctgacgcaacccccactggttggggcattgccaccacctgtcagctcctttccgggactttcgctttccccctccctattgccacggcggaactcatcgccgcctgccttgcccgctgctggacaggggctcggctgttgggcactgacaattccgtggtgttgtcggggaaatcatcgtcctttccttggctgctcgcctgtgttgccacctggattctgcgcgggacgtccttctgctacgtcccttcggccctcaatccagcggaccttccttcccgcggcctgctgccggctctgcggcctcttccgcgtcttcgccttcgccctcagacgagtcggatctccctttgggccgcctccccgcatcgataccgtcgactagccgtacctttaagaccaatgacttacaaggcagctgtagatcttagccactttttaaaagaaaaggggggactggaagggctaattcactcccaaagaagacaagatctgctttttgcctgtactgggtctctctggttagaccagatctgagcctgggagctctctggctaactagggaacccactgcttaagcctcaataaagcttgccttgagtgcttcaagtagtgtgtgcccgtctgttgtgtgactctggtaactagagatccctcagacccttttagtcagtgtggaaaatctctagcagaattcgatatcaagcttatcgataccgtcgacctcgagggggggcccggtacccaattcgccctatagtgagtcgtattacaattcactggccgtcgttttacaacgtcgtgactgggaaaaccctggcgttacccaacttaatcgccttgcagcacatccccctttcgccagctggcgtaatagcgaagaggcccgcaccgatcgcccttcccaacagttgcgcagcctgaatggcgaatggaaattgtaagcgttaatattttgttaaaattcgcgttaaatttttgttaaatcagctcattttttaaccaataggccgaaatcggcaaaatcccttataaatcaaaagaatagaccgagatagggttgagtgttgttccagtttggaacaagagtccactattaaagaacgtggactccaacgtcaaagggcgaaaaaccgtctatcagggcgatggcccactacgtgaaccatcaccctaatcaagttttttggggtcgaggtgccgtaaagcactaaatcggaaccctaaagggagcccccgatttagagcttgacggggaaagccggcgaacgtggcgagaaaggaagggaagaaagcgaaaggagcgggcgctagggcgctggcaagtgtagcggtcacgctgcgcgtaaccaccacacccgccgcgcttaatgcgccgctacagggcgcgtcaggtggcacttttcggggaaatgtgcgcggaacccctatttgtttatttttctaaatacattcaaatatgtatccgctcatgagacaataaccctgataaatgcttcaataatattgaaaaaggaagagtatgagtattcaacatttccgtgtcgcccttattcccttttttgcggcattttgccttcctgtttttgctcacccagaaacgctggtgaaagtaaaagatgctgaagatcagttgggtgcacgagtgggttacatcgaactggatctcaacagcggtaagatccttgagagttttcgccccgaagaacgttttccaatgatgagcacttttaaagttctgctatgtggcgcggtattatcccgtattgacgccgggcaagagcaactcggtcgccgcatacactattctcagaatgacttggttgagtactcaccagtcacagaaaagcatcttacggatggcatgacagtaagagaattatgcagtgctgccataaccatgagtgataacactgcggccaacttacttctgacaacgatcggaggaccgaaggagctaaccgcttttttgcacaacatgggggatcatgtaactcgccttgatcgttgggaaccggagctgaatgaagccataccaaacgacgagcgtgacaccacgatgcctgtagcaatggcaacaacgttgcgcaaactattaactggcgaactacttactctagcttcccggcaacaattaatagactggatggaggcggataaagttgcaggaccacttctgcgctcggcccttccggctggctggtttattgctgataaatctggagccggtgagcgtgggtctcgcggtatcattgcagcactggggccagatggtaagccctcccgtatcgtagttatctacacgacggggagtcaggcaactatggatgaacgaaatagacagatcgctgagataggtgcctcactgattaagcattggtaactgtcagaccaagtttactcatatatactttagattgatttaaaacttcatttttaatttaaaaggatctaggtgaagatcctttttgataatctcatgaccaaaatcccttaacgtgagttttcgttccactgagcgtcagaccccgtagaaaagatcaaaggatcttcttgagatcctttttttctgcgcgtaatctgctgcttgcaaacaaaaaaaccaccgctaccagcggtggtttgtttgccggatcaagagctaccaactctttttccgaaggtaactggcttcagcagagcgcagataccaaatactgttcttctagtgtagccgtagttaggccaccacttcaagaactctgtagcaccgcctacatacctcgctctgctaatcctgttaccagtggctgctgccagtggcgataagtcgtgtcttaccgggttggactcaagacgatagttaccggataaggcgcagcggtcgggctgaacggggggttcgtgcacacagcccagcttggagcgaacgacctacaccgaactgagatacctacagcgtgagctatgagaaagcgccacgcttcccgaagggagaaaggcggacaggtatccggtaagcggcagggtcggaacaggagagcgcacgagggagcttccagggggaaacgcctggtatctttatagtcctgtcgggtttcgccacctctgacttgagcgtcgatttttgtgatgctcgtcaggggggcggagcctatggaaaaacgccagcaacgcggcctttttacggttcctggccttttgctggccttttgctcacatgttctttcctgcgttatcccctgattctgtggataaccgtattaccgcctttgagtgagctgataccgctcgccgcagccgaacgaccgagcgcagcgagtcagtgagcgaggaagcggaagagcgcccaatacgcaaaccgcctctccccgcgcgttggccgattcattaatgcagctggcacgacaggtttcccgactggaaagcgggcagtgagcgcaacgcaattaatgtgagttagctcactcattaggcaccccaggctttacactttatgcttccggctcgtatgttgtgtggaattgtgagcggataacaatttcacacaggaaacagctatgaccatgattacgccaagctcgaaattaaccctcactaaagggaacaaaagctggagctccaccgcggtggcggcctcgaggtcgagatccggtcgaccagcaaccatagtcccgcccctaactccgcccatcccgcccctaactccgcccagttccgcccattctccgccccatggctgactaattttttttatttatgcagaggccgaggccgcctcggcctctgagctattccagaagtagtgaggaggcttttttggaggcctaggcttttgcaaaaagcttcgacggtatcgattggctcatgtccaacattaccgccatgttgacattgattattgactagttattaatagtaatcaattacggggtcattagttcatagcccatatatggagttccgcgttacataacttacggtaaatggcccgcctggctgaccgcccaacgacccccgcccattgacgtcaataatgacgtatgttcccatagtaacgccaatagggactttccattgacgtcaatgggtggagtatttacggtaaactgcccacttggcagtacatcaagtgtatcatatgccaagtacgccccctattgacgtcaatgacggtaaatggcccgcctggcattatgcccagtacatgaccttatgggactttcctacttggcagtacatctacgtattagtcatcgctattaccatggtgatgcggttttggcagtacatcaatgggcgtggatagcggtttgactcacggggatttccaagtctccaccccattgacgtcaatgggagtttgttttggcaccaaaatcaacgggactttccaaaatgtcgtaacaactccgccccattgacgcaaatgggcggtaggcgtgtacggaattcggagtggcgagccctcagatcctgcatataagcagctgctttttgcctgtactgggtctctctg

SEQ ID NO: 40 - protein, 952 aa, synthetic construct
  REGION 1..952: note = Synthetic
MLLLVTSLLLCELPHPAFLLIPQEQLVESGGRLVTPGGSLTLSCKASGFDFSAYYMSWVRQAPGKGLEWIATIYPSSGKTYYATWVNGRFTISSDNAQNTVDLQMNSLTAADRATYFCARDSYADDGALFNIWGPGTLVTISSGGGGSGGGGSGGGGSELVLTQSPSVSAALGSPAKITCTLSSAHKTDTIDWYQQLQGEAPRYLMQVQSDGSYTKRPGVPDRFSGSSSGADRYLIIPSVQADDEADYYCGADYIGGYVFGGGTQLTVTGESKYGPPCPPCPGQPREPQVYTLPPSQEEMTKNQVSLTCLVKGFYPSDIAVEWESNGQPENNYKTTPPVLDSDGSFFLYSRLTVDKSRWQEGNVFSCSVMHEALHNHYTQKSLSLSLGKMFWVLVVVGGVLACYSLLVTVAFIIFWVKRGRKKLLYIFKQPFMRPVQTTQEEDGCSCRFPEEEEGGCELRVKFSRSADAPAYQQGQNQLYNELNLGRREEYDVLDKRRGRDPEMGGKPRRKNPQEGLYNELQKDKMAEAYSEIGMKGERRRGKGHDGLYQGLSTATKDTYDALHMQALPPRLEGGGEGRGSLLTCGDVEENPGPRMLLLVTSLLLCELPHPAFLLIPRKVCNGIGIGEFKDSLSINATNIKHFKNCTSISGDLHILPVAFRGDSFTHTPPLDPQELDILKTVKEITGFLLIQAWPENRTDLHAFENLEIIRGRTKQHGQFSLAVVSLNITSLGLRSLKEISDGDVIISGNKNLCYANTINWKKLFGTSGQKTKIISNRGENSCKATGQVCHALCSPEGCWGPEPRDCVSCRNVSRGRECVDKCNLLEGEPREFVENSECIQCHPECLPQAMNITCTGRGPDNCIQCAHYIDGPHCVKTCPAGVMGENNTLVWKYADAGHVCHLCHPNCTYGCTGPGLEGCPTNGPKIPSIATGMVGALLLLLVVALGIGLFM

SEQ ID NO: 41 - DNA, 9400 bp, synthetic construct
  misc_feature 1..9400: note = Synthetic
  source 1..9400: mol_type = other DNA
gttagaccagatctgagcctgggagctctctggctaactagggaacccactgcttaagcctcaataaagcttgccttgagtgcttcaagtagtgtgtgcccgtctgttgtgtgactctggtaactagagatccctcagacccttttagtcagtgtggaaaatctctagcagtggcgcccgaacagggacttgaaagcgaaagggaaaccagaggagctctctcgacgcaggactcggcttgctgaagcgcgcacggcaagaggcgaggggcggcgactggtgagtacgccaaaaattttgactagcggaggctagaaggagagagatgggtgcgagagcgtcagtattaagcgggggagaattagatcgatgggaaaaaattcggttaaggccagggggaaagaaaaaatataaattaaaacatatagtatgggcaagcagggagctagaacgattcgcagttaatcctggcctgttagaaacatcagaaggctgtagacaaatactgggacagctacaaccatcccttcagacaggatcagaagaacttagatcattatataatacagtagcaaccctctattgtgtgcatcaaaggatagagataaaagacaccaaggaagctttagacaagatagaggaagagcaaaacaaaagtaagaaaaaagcacagcaagcagcagctgacacaggacacagcaatcaggtcagccaaaattaccctatagtgcagaacatccaggggcaaatggtacatcaggccatatcacctagaactttaaatgcatgggtaaaagtagtagaagagaaggctttcagcccagaagtgatacccatgttttcagcattatcagaaggagccaccccacaagatttaaacaccatgctaaacacagtggggggacatcaagcagccatgcaaatgttaaaagagaccatcaatgaggaagctgcaggcaaagagaagagtggtgcagagagaaaaaagagcagtgggaataggagctttgttccttgggttcttgggagcagcaggaagcactatgggcgcagcgtcaatgacgctgacggtacaggccagacaattattgtctggtatagtgcagcagcagaacaatttgctgagggctattgaggcgcaacagcatctgttgcaactcacagtctggggcatcaagcagctccaggcaagaatcctggctgtggaaagatacctaaaggatcaacagctcctggggatttggggttgctctggaaaactcatttgcaccactgctgtgccttggatctacaaatggcagtattcatccacaattttaaaagaaaaggggggattggggggtacagtgcaggggaaagaatagtagacataatagcaacagacatacaaactaaagaattacaaaaacaaattacaaaaattcaaaattttcgggtttattacagggacagcagagatccagtttggggatcaattgcatgaagaatctgcttagggttaggcgttttgcgctgcttcgcgaggatctgcgatcgctccggtgcccgtcagtgggcagagcgcacatcgcccacagtccccgagaagttggggggaggggtcggcaattgaaccggtgcctagagaaggtggcgcggggtaaactgggaaagtgatgtcgtgtactggctccgcctttttcccgagggtgggggagaaccgtatataagtgcagtagtcgccgtgaacgttctttttcgcaacgggtttgccgccagaacacagctgaagcttcgaggggctcgcatctctccttcacgcgcccgccgccctacctgaggccgccatccacgccggttgagtcgcgttctgccgcctcccgcctgtggtgcctcctgaactgcgtccgccgtctaggtaagtttaaagctcaggtcgagaccgggcctttgtccggcgctcccttggagcctacctagactcagccggctctccacgctttgcctgaccctgcttgctcaactctacgtctttgtttcgttttctgttctgcgccgttacagatccaagctgtgaccggcgcctacggctagcgaattcctcgaggccaccatgctgctgctggtgacaagcctgctgctgtgcgagctgccccaccccgcctttctgctgatcccccaggaacagctcgtcgaaagcggcggcagactggtgacacctggcggcagcctgaccctgagctgcaaggccagcggcttcgacttcagcgcctactacatgagctgggtccgccaggcccctggcaagggactggaatggatcgccaccatctaccccagcagcggcaagacctactacgccacctgggtgaacggacggttcaccatctccagcgacaacgcccagaacaccgtggacctgcagatgaacagcctgacagccgccgaccgggccacctacttttgcgccagagacagctacgccgacgacggcgccctgttcaacatctggggccctggcaccctggtgacaatctctagcggcggaggcggatctggtggcggaggaagtggcggcggaggatctgagctggtgctgacccagagcccctctgtgtctgctgccctgggaagccctgccaagatcacctgtaccctgagcagcgcccacaagaccgacaccatcgactggtatcagcagctgcagggcgaggcccccagatacctgatgcaggtgcagagcgacggcagctacaccaagaggccaggcgtgcccgaccggttcagcggatctagctctggcgccgaccgctacctgatcatccccagcgtgcaggccgatgacgaggccgattactactgtggcgccgactacatcggcggctacgtgttcggcggaggcacccagctgaccgtgaccggcgagtctaagtacggaccgccctgccccccttgccctatgttctgggtgctggtggtggtgggcggggtgctggcctgctacagcctgctggtgacagtggccttcatcatcttttgggtgaaacggggcagaaagaaactcctgtatatattcaaacaaccatttatgagaccagtacaaactactcaagaggaagatggctgtagctgccgatttccagaagaagaagaaggaggatgtgaactgcgggtgaagttcagcagaagcgccgacgcccctgcctaccagcagggccagaatcagctgtacaacgagctgaacctgggcagaagggaagagtacgacgtcctggataagcggagaggccgggaccctgagatgggcggcaagcctcggcggaagaacccccaggaaggcctgtataacgaactgcagaaagacaagatggccgaggcctacagcgagatcggcatgaagggcgagcggaggcggggcaagggccacgacggcctgtatcagggcctgtccaccgccaccaaggatacctacgacgccctgcacatgcaggccctgcccccaaggctcgagggcggcggagagggcagaggaagtcttctaacatgcggtgacgtggaggagaatcccggccctaggatgcttctcctggtgacaagccttctgctctgtgagttaccacacccagcattcctcctgatcccacgcaaagtgtgtaacggaataggtattggtgaatttaaagactcactctccataaatgctacgaatattaaacacttcaaaaactgcacctccatcagtggcgatctccacatcctgccggtggcatttaggggtgactccttcacacatactcctcctctggatccacaggaactggatattctgaaaaccgtaaaggaaatcacagggtttttgctgattcaggcttggcctgaaaacaggacggacctccatgcctttgagaacctagaaatcatacgcggcaggaccaagcaacatggtcagttttctcttgcagtcgtcagcctgaacataacatccttgggattacgctccctcaaggagataagtgatggagatgtgataatttcaggaaacaaaaatttgtgctatgcaaatacaataaactggaaaaaactgtttgggacctccggtcagaaaaccaaaattataagcaacagaggtgaaaacagctgcaaggccacaggccaggtctgccatgccttgtgctcccccgagggctgctggggcccggagcccagggactgcgtctcttgccggaatgtcagccgaggcagggaatgcgtggacaagtgcaaccttctggagggtgagccaagggagtttgtggagaactctgagtgcatacagtgccacccagagtgcctgcctcaggccatgaacatcacctgcacaggacggggaccagacaactgtatccagtgtgcccactacattgacggcccccactgcgtcaagacctgcccggcaggagtcatgggagaaaacaacaccctggtctggaagtacgcagacgccggccatgtgtgccacctgtgccatccaaactgcacctacggatgcactgggccaggtcttgaaggctgtccaacgaatgggcctaagatcccgtccatcgccactgggatggtgggggccctcctcttgctgctggtggtggccctggggatcggcctcttcatgtgagcggccgctctagacccgggctgcaggaattcgatatcaagcttatcgataatcaacctctggattacaaaatttgtgaaagattgactggtattcttaactatgttgctccttttacgctatgtggatacgctgctttaatgcctttgtatcatgctattgcttcccgtatggctttcattttctcctccttgtataaatcctggttgctgtctctttatgaggagttgtggcccgttgtcaggcaacgtggcgtggtgtgcactgtgtttgctgacgcaacccccactggttggggcattgccaccacctgtcagctcctttccgggactttcgctttccccctccctattgccacggcggaactcatcgccgcctgccttgcccgctgctggacaggggctcggctgttgggcactgacaattccgtggtgttgtcggggaaatcatcgtcctttccttggctgctcgcctgtgttgccacctggattctgcgcgggacgtccttctgctacgtcccttcggccctcaatccagcggaccttccttcccgcggcctgctgccggctctgcggcctcttccgcgtcttcgccttcgccctcagacgagtcggatctccctttgggccgcctccccgcatcgataccgtcgactagccgtacctttaagaccaatgacttacaaggcagctgtagatcttagccactttttaaaagaaaaggggggactggaagggctaattcactcccaaagaagacaagatctgctttttgcctgtactgggtctctctggttagaccagatctgagcctgggagctctctggctaactagggaacccactgcttaagcctcaataaagcttgccttgagtgcttcaagtagtgtgtgcccgtctgttgtgtgactctggtaactagagatccctcagacccttttagtcagtgtggaaaatctctagcagaattcgatatcaagcttatcgataccgtcgacctcgagggggggcccggtacccaattcgccctatagtgagtcgtattacaattcactggccgtcgttttacaacgtcgtgactgggaaaaccctggcgttacccaacttaatcgccttgcagcacatccccctttcgccagctggcgtaatagcgaagaggcccgcaccgatcgcccttcccaacagttgcgcagcctgaatggcgaatggaaattgtaagcgttaatattttgttaaaattcgcgttaaatttttgttaaatcagctcattttttaaccaataggccgaaatcggcaaaatcccttataaatcaaaagaatagaccgagatagggttgagtgttgttccagtttggaacaagagtccactattaaagaacgtggactccaacgtcaaagggcgaaaaaccgtctatcagggcgatggcccactacgtgaaccatcaccctaatcaagttttttggggtcgaggtgccgtaaagcactaaatcggaaccctaaagggagcccccgatttagagcttgacggggaaagccggcgaacgtggcgagaaaggaagggaagaaagcgaaaggagcgggcgctagggcgctggcaagtgtagcggtcacgctgcgcgtaaccaccacacccgccgcgcttaatgcgccgctacagggcgcgtcaggtggcacttttcggggaaatgtgcgcggaacccctatttgtttatttttctaaatacattcaaatatgtatccgctcatgagacaataaccctgataaatgcttcaataatattgaaaaaggaagagtatgagtattcaacatttccgtgtcgcccttattcccttttttgcggcattttgccttcctgtttttgctcacccagaaacgctggtgaaagtaaaagatgctgaagatcagttgggtgcacgagtgggttacatcgaactggatctcaacagcggtaagatccttgagagttttcgccccgaagaacgttttccaatgatgagcacttttaaagttctgctatgtggcgcggtattatcccgtattgacgccgggcaagagcaactcggtcgccgcatacactattctcagaatgacttggttgagtactcaccagtcacagaaaagcatcttacggatggcatgacagtaagagaattatgcagtgctgccataaccatgagtgataacactgcggccaacttacttctgacaacgatcggaggaccgaaggagctaaccgcttttttgcacaacatgggggatcatgtaactcgccttgatcgttgggaaccggagctgaatgaagccataccaaacgacgagcgtgacaccacgatgcctgtagcaatggcaacaacgttgcgcaaactattaactggcgaactacttactctagcttcccggcaacaattaatagactggatggaggcggataaagttgcaggaccacttctgcgctcggcccttccggctggctggtttattgctgataaatctggagccggtgagcgtgggtctcgcggtatcattgcagcactggggccagatggtaagccctcccgtatcgtagttatctacacgacggggagtcaggcaactatggatgaacgaaatagacagatcgctgagataggtgcctcactgattaagcattggtaactgtcagaccaagtttactcatatatactttagattgatttaaaacttcatttttaatttaaaaggatctaggtgaagatcctttttgataatctcatgaccaaaatcccttaacgtgagttttcgttccactgagcgtcagaccccgtagaaaagatcaaaggatcttcttgagatcctttttttctgcgcgtaatctgctgcttgcaaacaaaaaaaccaccgctaccagcggtggtttgtttgccggatcaagagctaccaactctttttccgaaggtaactggcttcagcagagcgcagataccaaatactgttcttctagtgtagccgtagttaggccaccacttcaagaactctgtagcaccgcctacatacctcgctctgctaatcctgttaccagtggctgctgccagtggcgataagtcgtgtcttaccgggttggactcaagacgatagttaccggataaggcgcagcggtcgggctgaacggggggttcgtgcacacagcccagcttggagcgaacgacctacaccgaactgagatacctacagcgtgagctatgagaaagcgccacgcttcccgaagggagaaaggcggacaggtatccggtaagcggcagggtcggaacaggagagcgcacgagggagcttccagggggaaacgcctggtatctttatagtcctgtcgggtttcgccacctctgacttgagcgtcgatttttgtgatgctcgtcaggggggcggagcctatggaaaaacgccagcaacgcggcctttttacggttcctggccttttgctggccttttgctcacatgttctttcctgcgttatcccctgattctgtggataaccgtattaccgcctttgagtgagctgataccgctcgccgcagccgaacgaccgagcgcagcgagtcagtgagcgaggaagcggaagagcgcccaatacgcaaaccgcctctccccgcgcgttggccgattcattaatgcagctggcacgacaggtttcccgactggaaagcgggcagtgagcgcaacgcaattaatgtgagttagctcactcattaggcaccccaggctttacactttatgcttccggctcgtatgttgtgtggaattgtgagcggataacaatttcacacaggaaacagctatgaccatgattacgccaagctcgaaattaaccctcactaaagggaacaaaagctggagctccaccgcggtggcggcctcgaggtcgagatccggtcgaccagcaaccatagtcccgcccctaactccgcccatcccgcccctaactccgcccagttccgcccattctccgccccatggctgactaattttttttatttatgcagaggccgaggccgcctcggcctctgagctattccagaagtagtgaggaggcttttttggaggcctaggcttttgcaaaaagcttcgacggtatcgattggctcatgtccaacattaccgccatgttgacattgattattgactagttattaatagtaatcaattacggggtcattagttcatagcccatatatggagttccgcgttacataacttacggtaaatggcccgcctggctgaccgcccaacgacccccgcccattgacgtcaataatgacgtatgttcccatagtaacgccaatagggactttccattgacgtcaatgggtggagtatttacggtaaactgcccacttggcagtacatcaagtgtatcatatgccaagtacgccccctattgacgtcaatgacggtaaatggcccgcctggcattatgcccagtacatgaccttatgggactttcctacttggcagtacatctacgtattagtcatcgctattaccatggtgatgcggttttggcagtacatcaatgggcgtggatagcggtttgactcacggggatttccaagtctccaccccattgacgtcaatgggagtttgttttggcaccaaaatcaacgggactttccaaaatgtcgtaacaactccgccccattgacgcaaatgggcggtaggcgtgtacggaattcggagtggcgagccctcagatcctgcatataagcagctgctttttgcctgtactgggtctctctg

SEQ ID NO: 42 - protein, 845 aa, synthetic construct
  REGION 1..845: note = Synthetic
MLLLVTSLLLCELPHPAFLLIPQEQLVESGGRLVTPGGSLTLSCKASGFDFSAYYMSWVRQAPGKGLEWIATIYPSSGKTYYATWVNGRFTISSDNAQNTVDLQMNSLTAADRATYFCARDSYADDGALFNIWGPGTLVTISSGGGGSGGGGSGGGGSELVLTQSPSVSAALGSPAKITCTLSSAHKTDTIDWYQQLQGEAPRYLMQVQSDGSYTKRPGVPDRFSGSSSGADRYLIIPSVQADDEADYYCGADYIGGYVFGGGTQLTVTGESKYGPPCPPCPMFWVLVVVGGVLACYSLLVTVAFIIFWVKRGRKKLLYIFKQPFMRPVQTTQEEDGCSCRFPEEEEGGCELRVKFSRSADAPAYQQGQNQLYNELNLGRREEYDVLDKRRGRDPEMGGKPRRKNPQEGLYNELQKDKMAEAYSEIGMKGERRRGKGHDGLYQGLSTATKDTYDALHMQALPPRLEGGGEGRGSLLTCGDVEENPGPRMLLLVTSLLLCELPHPAFLLIPRKVCNGIGIGEFKDSLSINATNIKHFKNCTSISGDLHILPVAFRGDSFTHTPPLDPQELDILKTVKEITGFLLIQAWPENRTDLHAFENLEIIRGRTKQHGQFSLAVVSLNITSLGLRSLKEISDGDVIISGNKNLCYANTINWKKLFGTSGQKTKIISNRGENSCKATGQVCHALCSPEGCWGPEPRDCVSCRNVSRGRECVDKCNLLEGEPREFVENSECIQCHPECLPQAMNITCTGRGPDNCIQCAHYIDGPHCVKTCPAGVMGENNTLVWKYADAGHVCHLCHPNCTYGCTGPGLEGCPTNGPKIPSIATGMVGALLLLLVVALGIGLFM

SEQ ID NO: 43 - DNA, 10015 bp, synthetic construct
  misc_feature 1..10015: note = Synthetic
  source 1..10015: mol_type = other DNA
gttagaccagatctgagcctgggagctctctggctaactagggaacccactgcttaagcctcaataaagcttgccttgagtgcttcaagtagtgtgtgcccgtctgttgtgtgactctggtaactagagatccctcagacccttttagtcagtgtggaaaatctctagcagtggcgcccgaacagggacttgaaagcgaaagggaaaccagaggagctctctcgacgcaggactcggcttgctgaagcgcgcacggcaagaggcgaggggcggcgactggtgagtacgccaaaaattttgactagcggaggctagaaggagagagatgggtgcgagagcgtcagtattaagcgggggagaattagatcgatgggaaaaaattcggttaaggccagggggaaagaaaaaatataaattaaaacatatagtatgggcaagcagggagctagaacgattcgcagttaatcctggcctgttagaaacatcagaaggctgtagacaaatactgggacagctacaaccatcccttcagacaggatcagaagaacttagatcattatataatacagtagcaaccctctattgtgtgcatcaaaggatagagataaaagacaccaaggaagctttagacaagatagaggaagagcaaaacaaaagtaagaaaaaagcacagcaagcagcagctgacacaggacacagcaatcaggtcagccaaaattaccctatagtgcagaacatccaggggcaaatggtacatcaggccatatcacctagaactttaaatgcatgggtaaaagtagtagaagagaaggctttcagcccagaagtgatacccatgttttcagcattatcagaaggagccaccccacaagatttaaacaccatgctaaacacagtggggggacatcaagcagccatgcaaatgttaaaagagaccatcaatgaggaagctgcaggcaaagagaagagtggtgcagagagaaaaaagagcagtgggaataggagctttgttccttgggttcttgggagcagcaggaagcactatgggcgcagcgtcaatgacgctgacggtacaggccagacaattattgtctggtatagtgcagcagcagaacaatttgctgagggctattgaggcgcaacagcatctgttgcaactcacagtctggggcatcaagcagctccaggcaagaatcctggctgtggaaagatacctaaaggatcaacagctcctggggatttggggttgctctggaaaactcatttgcaccactgctgtgccttggatctacaaatggcagtattcatccacaattttaaaagaaaaggggggattggggggtacagtgcaggggaaagaatagtagacataatagcaacagacatacaaactaaagaattacaaaaacaaattacaaaaattcaaaattttcgggtttattacagggacagcagagatccagtttggggatcaattgcatgaagaatctgcttagggttaggcgttttgcgctgcttcgcgaggatctgcgatcgctccggtgcccgtcagtgggcagagcgcacatcgcccacagtccccgagaagttggggggaggggtcggcaattgaaccggtgcctagagaaggtggcgcggggtaaactgggaaagtgatgtcgtgtactggctccgcctttttcccgagggtgggggagaaccgtatataagtgcagtagtcgccgtgaacgttctttttcgcaacgggtttgccgccagaacacagctgaagcttcgaggggctcgcatctctccttcacgcgcccgccgccctacctgaggccgccatccacgccggttgagtcgcgttctgccgcctcccgcctgtggtgcctcctgaactgcgtccgccgtctaggtaagtttaaagctcaggtcgagaccgggcctttgtccggcgctcccttggagcctacctagactcagccggctctccacgctttgcctgaccctgcttgctcaactctacgtctttgtttcgttttctgttctgcgccgttacagatccaagctgtgaccggcgcctacggctagcgaattcgccaccatgctgctgctggtgacaagcctgctgctgtgcgagctgccccaccccgcctttctgctgatcccccagagcgtgaaagagtccgagggcgacctggtcacaccagccggcaacctgaccctgacctgtaccgccagcggcagcgacatcaacgactaccccatctcttgggtccgccaggctcctggcaagggactggaatggatcggcttcatcaacagcggcggcagcacttggtacgccagctgggtcaaaggccggttcaccatcagccggaccagcaccaccgtggacctgaagatgacaagcctgaccaccgacgacaccgccacctacttttgcgccagaggctacagcacctactacggcgacttcaacatctggggccctggcaccctggtcacaatctctagcggcggaggcggcagcggaggtggaggaagtggcggcggaggatccgagctggtcatgacccagacccccagcagcacatctggcgccgtgggcggcaccgtgaccatcaattgccaggccagccagagcatcgacagcaacctggcctggttccagcagaagcccggccagccccccaccctgctgatctacagagcctccaacctggccagcggcgtgccaagcagattcagcggcagcagatctggcaccgagtacaccctgaccatctccggcgtgcagagagaggacgccgctacctattactgcctgggcggcgtgggcaacgtgtcctacagaaccagcttcggcggaggtactgaggtggtcgtcaaatacggaccgccctgccccccttgccctgcccccgagttcctgggcggacccagcgtgttcctgttcccccccaagcccaaggacaccctgatgatcagccggacccccgaggtgacctgcgtggtggtggacgtgagccaggaagatcccgaggtccagttcaattggtacgtggacggcgtggaagtgcacaacgccaagaccaagcccagagaggaacagttcaacagcacctaccgggtggtgtctgtgctgaccgtgctgcaccaggactggctgaacggcaaagaatacaagtgcaaggtgtccaacaagggcctgcccagcagcatcgaaaagaccatcagcaaggccaagggccagcctcgcgagccccaggtgtacaccctgcctccctcccaggaagagatgaccaagaaccaggtgtccctgacctgcctggtgaagggcttctaccccagcgacatcgccgtggagtgggagagcaacggccagcctgagaacaactacaagaccacccctcccgtgctggacagcgacggcagcttcttcctgtacagccggctgaccgtggacaagagccggtggcaggaaggcaacgtctttagctgcagcgtgatgcacgaggccctgcacaaccactacacccagaagagcctgagcctgtccctgggcaagatgttctgggtgctggtggtggtgggcggggtgctggcctgctacagcctgctggtgacagtggccttcatcatcttttgggtgaaacggggcagaaagaaactcctgtatatattcaaacaaccatttatgagaccagtacaaactactcaagaggaagatggctgtagctgccgatttccagaagaagaagaaggaggatgtgaactgcgggtgaagttcagcagaagcgccgacgcccctgcctaccagcagggccagaatcagctgtacaacgagctgaacctgggcagaagggaagagtacgacgtcctggataagcggagaggccgggaccctgagatgggcggcaagcctcggcggaagaacccccaggaaggcctgtataacgaactgcagaaagacaagatggccgaggcctacagcgagatcggcatgaagggcgagcggaggcggggcaagggccacgacggcctgtatcagggcctgtccaccgccaccaaggatacctacgacgccctgcacatgcaggccctgcccccaaggctcgagggcggcggagagggcagaggaagtcttctaacatgcggtgacgtggaggagaatcccggccctaggatgcttctcctggtgacaagccttctgctctgtgagttaccacacccagcattcctcctgatcccacgcaaagtgtgtaacggaataggtattggtgaatttaaagactcactctccataaatgctacgaatattaaacacttcaaaaactgcacctccatcagtggcgatctccacatcctgccggtggcatttaggggtgactccttcacacatactcctcctctggatccacaggaactggatattctgaaaaccgtaaaggaaatcacagggtttttgctgattcaggcttggcctgaaaacaggacggacctccatgcctttgagaacctagaaatcatacgcggcaggaccaagcaacatggtcagttttctcttgcagtcgtcagcctgaacataacatccttgggattacgctccctcaaggagataagtgatggagatgtgataatttcaggaaacaaaaatttgtgctatgcaaatacaataaactggaaaaaactgtttgggacctccggtcagaaaaccaaaattataagcaacagaggtgaaaacagctgcaaggccacaggccaggtctgccatgccttgtgctcccccgagggctgctggggcccggagcccagggactgcgtctcttgccggaatgtcagccgaggcagggaatgcgtggacaagtgcaaccttctggagggtgagccaagggagtttgtggagaactctgagtgcatacagtgccacccagagtgcctgcctcaggccatgaacatcacctgcacaggacggggaccagacaactgtatccagtgtgcccactacattgacggcccccactgcgtcaagacctgcccggcaggagtcatgggagaaaacaacaccctggtctggaagtacgcagacgccggccatgtgtgccacctgtgccatccaaactgcacctacggatgcactgggccaggtcttgaaggctgtccaacgaatgggcctaagatcccgtccatcgccactgggatggtgggggccctcctcttgctgctggtggtggccctggggatcggcctcttcatgtgagcggccgctctagacccgggctgcaggaattcgatatcaagcttatcgataatcaacctctggattacaaaatttgtgaaagattgactggtattcttaactatgttgctccttttacgctatgtggatacgctgctttaatgcctttgtatcatgctattgcttcccgtatggctttcattttctcctccttgtataaatcctggttgctgtctctttatgaggagttgtggcccgttgtcaggcaacgtggcgtggtgtgcactgtgtttgctgacgcaacccccactggttggggcattgccaccacctgtcagctcctttccgggactttcgctttccccctccctattgccacggcggaactcatcgccgcctgccttgcccgctgctggacaggggctcggctgttgggcactgacaattccgtggtgttgtcggggaaatcatcgtcctttccttggctgctcgcctgtgttgccacctggattctgcgcgggacgtccttctgctacgtcccttcggccctcaatccagcggaccttccttcccgcggcctgctgccggctctgcggcctcttccgcgtcttcgccttcgccctcagacgagtcggatctccctttgggccgcctccccgcatcgataccgtcgactagccgtacctttaagaccaatgacttacaaggcagctgtagatcttagccactttttaaaagaaaaggggggactggaagggctaattcactcccaaagaagacaagatctgctttttgcctgtactgggtctctctggttagaccagatctgagcctgggagctctctggctaactagggaacccactgcttaagcctcaataaagcttgccttgagtgcttcaagtagtgtgtgcccgtctgttgtgtgactctggtaactagagatccctcagacccttttagtcagtgtggaaaatctctagcagaattcgatatcaagcttatcgataccgtcgacctcgagggggggcccggtacccaattcgccctatagtgagtcgtattacaattcactggccgtcgttttacaacgtcgtgactgggaaaaccctggcgttacccaacttaatcgccttgcagcacatccccctttcgccagctggcgtaatagcgaagaggcccgcaccgatcgcccttcccaacagttgcgcagcctgaatggcgaatggaaattgtaagcgttaatattttgttaaaattcgcgttaaatttttgttaaatcagctcattttttaaccaataggccgaaatcggcaaaatcccttataaatcaaaagaatagaccgagatagggttgagtgttgttccagtttggaacaagagtccactattaaagaacgtggactccaacgtcaaagggcgaaaaaccgtctatcagggcgatggcccactacgtgaaccatcaccctaatcaagttttttggggtcgaggtgccgtaaagcactaaatcggaaccctaaagggagcccccgatttagagcttgacggggaaagccggcgaacgtggcgagaaaggaagggaagaaagcgaaaggagcgggcgctagggcgctggcaagtgtagcggtcacgctgcgcgtaaccaccacacccgccgcgcttaatgcgccgctacagggcgcgtcaggtggcacttttcggggaaatgtgcgcggaacccctatttgtttatttttctaaatacattcaaatatgtatccgctcatgagacaataaccctgataaatgcttcaataatattgaaaaaggaagagtatgagtattcaacatttccgtgtcgcccttattcccttttttgcggcattttgccttcctgtttttgctcacccagaaacgctggtgaaagtaaaagatgctgaagatcagttgggtgcacgagtgggttacatcgaactggatctcaacagcggtaagatccttgagagttttcgccccgaagaacgttttccaatgatgagcacttttaaagttctgctatgtggcgcggtattatcccgtattgacgccgggcaagagcaactcggtcgccgcatacactattctcagaatgacttggttgagtactcaccagtcacagaaaagcatcttacggatggcatgacagtaagagaattatgcagtgctgccataaccatgagtgataacactgcggccaacttacttctgacaacgatcggaggaccgaaggagctaaccgcttttttgcacaacatgggggatcatgtaactcgccttgatcgttgggaaccggagctgaatgaagccataccaaacgacgagcgtgacaccacgatgcctgtagcaatggcaacaacgttgcgcaaactattaactggcgaactacttactctagcttcccggcaacaattaatagactggatggaggcggataaagttgcaggaccacttctgcgctcggcccttccggctggctggtttattgctgataaatctggagccggtgagcgtgggtctcgcggtatcattgcagcactggggccagatggtaagccctcccgtatcgtagttatctacacgacggggagtcaggcaactatggatgaacgaaatagacagatcgctgagataggtgcctcactgattaagcattggtaactgtcagaccaagtttactcatatatactttagattgatttaaaacttcatttttaatttaaaaggatctaggtgaagatcctttttgataatctcatgaccaaaatcccttaacgtgagttttcgttccactgagcgtcagaccccgtagaaaagatcaaaggatcttcttgagatcctttttttctgcgcgtaatctgctgcttgcaaacaaaaaaaccaccgctaccagcggtggtttgtttgccggatcaagagctaccaactctttttccgaaggtaactggcttcagcagagcgcagataccaaatactgttcttctagtgtagccgtagttaggccaccacttcaagaactctgtagcaccgcctacatacctcgctctgctaatcctgttaccagtggctgctgccagtggcgataagtcgtgtcttaccgggttggactcaagacgatagttaccggataaggcgcagcggtcgggctgaacggggggttcgtgcacacagcccagcttggagcgaacgacctacaccgaactgagatacctacagcgtgagctatgagaaagcgccacgcttcccgaagggagaaaggcggacaggtatccggtaagcggcagggtcggaacaggagagcgcacgagggagcttccagggggaaacgcctggtatctttatagtcctgtcgggtttcgccacctctgacttgagcgtcgatttttgtgatgctcgtcaggggggcggagcctatggaaaaacgccagcaacgcggcctttttacggttcctggccttttgctggccttttgctcacatgttctttcctgcgttatcccctgattctgtggataaccgtattaccgcctttgagtgagctgataccgctcgccgcagccgaacgaccgagcgcagcgagtcagtgagcgaggaagcggaagagcgcccaatacgcaaaccgcctctccccgcgcgttggccgattcattaatgcagctggcacgacaggtttcccgactggaaagcgggcagtgagcgcaacgcaattaatgtgagttagctcactcattaggcaccccaggctttacactttatgcttccggctcgtatgttgtgtggaattgtgagcggataacaatttcacacaggaaacagctatgaccatgattacgccaagctcgaaattaaccctcactaaagggaacaaaagctggagctccaccgcggtggcggcctcgaggtcgagatccggtcgaccagcaaccatagtcccgcccctaactccgcccatcccgcccctaactccgcccagttccgcccattctccgccccatggctgactaattttttttatttatgcagaggccgaggccgcctcggcctctgagctattccagaagtagtgaggaggcttttttggaggcctaggcttttgcaaaaagcttcgacggtatcgattggctcatgtccaacattaccgccatgttgacattgattattgactagttattaatagtaatcaattacggggtcattagttcatagcccatatatggagttccgcgttacataacttacggtaaatggcccgcctggctgaccgcccaacgacccccgcccattgacgtcaataatgacgtatgttcccatagtaacgccaatagggactttccattgacgtcaatgggtggagtatttacggtaaactgcccacttggcagtacatcaagtgtatcatatgccaagtacgccccctattgacgtcaatgacggtaaatggcccgcctggcattatgcccagtacatgaccttatgggactttcctacttggcagtacatctacgtattagtcatcgctattaccatggtgatgcggttttggcagtacatcaatgggcgtggatagcggtttgactcacggggatttccaagtctccaccccattgacgtcaatgggagtttgttttggcaccaaaatcaacgggactttccaaaatgtcgtaacaactccgccccattgacgcaaatgggcggtaggcgtgtacggaattcggagtggcgagccctcagatcctgcatataagcagctgctttttgcctgtactgggtctctctg

SEQ ID NO: 44 - protein, 1055 aa, synthetic construct [sequence omitted]

SEQ ID NO: 45 - DNA, 10015 bp, synthetic construct; identical to SEQ ID NO: 43
  misc_feature 1..10015: note = Synthetic
  source 1..10015: mol_type = other DNA

SEQ ID NO: 46 - protein, 945 aa, synthetic construct
  REGION 1..945: note = Synthetic
MLLLVTSLLLCELPHPAFLLIPQSVKESEGDLVTPAGNLTLTCTASGSDINDYPISWVRQAPGKGLEWIGFINSGGSTWYASWVKGRFTISRTSTTVDLKMTSLTTDDTATYFCARGYSTYYGDFNIWGPGTLVTISSGGGGSGGGGSGGGGSELVMTQTPSSTSGAVGGTVTINCQASQSIDSNLAWFQQKPGQPPTLLIYRASNLASGVPSRFSGSRSGTEYTLTISGVQREDAATYYCLGGVGNVSYRTSFGGGTEVVVKESKYGPPCPPCPGQPREPQVYTLPPSQEEMTKNQVSLTCLVKGFYPSDIAVEWESNGQPENNYKTTPPVLDSDGSFFLYSRLTVDKSRWQEGNVFSCSVMHEALHNHYTQKSLSLSLGKMFWVLVVVGGVLACYSLLVTVAFIIFWVKRGRKKLLYIFKQPFMRPVQTTQEEDGCSCRFPEEEEGGCELRVKFSRSADAPAYQQGQNQLYNELNLGRREEYDVLDKRRGRDPEMGGKPRRKNPQEGLYNELQKDKMAEAYSEIGMKGERRRGKGHDGLYQGLSTATKDTYDALHMQALPPRLEGGGEGRGSLLTCGDVEENPGPRMLLLVTSLLLCELPHPAFLLIPRKVCNGIGIGEFKDSLSINATNIKHFKNCTSISGDLHILPVAFRGDSFTHTPPLDPQELDILKTVKEITGFLLIQAWPENRTDLHAFENLEIIRGRTKQHGQFSLAVVSLNITSLGLRSLKEISDGDVIISGNKNLCYANTINWKKLFGTSGQKTKIISNRGENSCKATGQVCHALCSPEGCWGPEPRDCVSCRNVSRGRECVDKCNLLEGEPREFVENSECIQCHPECLPQAMNITCTGRGPDNCIQCAHYIDGPHCVKTCPAGVMGENNTLVWKYADAGHVCHLCHPNCTYGCTGPGLEGCPTNGPKIPSIATGMVGALLLLLVVALGIGLFM

SEQ ID NO: 47 - DNA, 9685 bp, synthetic construct
  misc_feature 1..9685: note = Synthetic
  source 1..9685: mol_type = other DNA
gttagaccagatctgagcctgggagctctctggctaactagggaacccactgcttaagcctcaataaagcttgccttgagtgcttcaagtagtgtgtgcccgtctgttgtgtgactctggtaactagagatccctcagacccttttagtcagtgtggaaaatctctagcagtggcgcccgaacagggacttgaaagcgaaagggaaaccagaggagctctctcgacgcaggactcggcttgctgaagcgcgcacggcaagaggcgaggggcggcgactggtgagtacgccaaaaattttgactagcggaggctagaaggagagagatgggtgcgagagcgtcagtattaagcgggggagaattagatcgatgggaaaaaattcggttaaggccagggggaaagaaaaaatataaattaaaacatatagtatgggcaagcagggagctagaacgattcgcagttaatcctggcctgttagaaacatcagaaggctgtagacaaatactgggacagctacaaccatcccttcagacaggatcagaagaacttagatcattatataatacagtagcaaccctctattgtgtgcatcaaaggatagagataaaagacaccaaggaagctttagacaagatagaggaagagcaaaacaaaagtaagaaaaaagcacagcaagcagcagctgacacaggacacagcaatcaggtcagccaaaattaccctatagtgcagaacatccaggggcaaatggtacatcaggccatatcacctagaactttaaatgcatgggtaaaagtagtagaagagaaggctttcagcccagaagtgatacccatgttttcagcattatcagaaggagccaccccacaagatttaaacaccatgctaaacacagtggggggacatcaagcagccatgcaaatgttaaaagagaccatcaatgaggaagctgcaggcaaagagaagagtggtgcagagagaaaaaagagcagtgggaataggagctttgttccttgggttcttgggagcagcaggaagcactatgggcgcagcgtcaatgacgctgacggtacaggccagacaattattgtctggtatagtgcagcagcagaacaatttgctgagggctattgaggcgcaacagcatctgttgcaactcacagtctggggcatcaagcagctccaggcaagaatcctggctgtggaaagatacctaaaggatcaacagctcctggggatttggggttgctctggaaaactcatttgcaccactgctgtgccttggatctacaaatggcagtattcatccacaattttaaaagaaaaggggggattggggggtacagtgcaggggaaagaatagtagacataatagcaacagacatacaaactaaagaattacaaaaacaaattacaaaaattcaaaattttcgggtttattacagggacagcagagatccagtttggggatcaattgcatgaagaatctgcttagggttaggcgttttgcgctgcttcgcgaggatctgcgatcgctccggtgcccgtcagtgggcagagcgcacatcgcccacagtccccgagaagttggggggaggggtcggcaattgaaccggtgcctagagaaggtggcgcggggtaaactgggaaagtgatgtcgtgtactggctccgcctttttcccgagggtgggggagaaccgtatataagtgcagtagtcgccgtgaacgttctttttcgcaacgggtttgccgccagaacacagctgaagcttcgaggggctcgcatctctccttcacgcgcccgccgccctacctgaggccgccatccacgccggttgagtcgcgttctgccgcctcccgcctgtggtgcctcctgaactgcgtccgccgtctaggtaagtttaaagctcaggtcgagaccgggcctttgtccggcgctcccttggagcctacctagactcagccggctctccacgctttgcctgaccctgcttgctcaactctacgtctttgtttcgttttctgttctgcgccgttacagatccaagctgtgaccggcgcctacggctagcgaattcgccaccatgctgctgctggtgacaagcctgctgctgtgcgagctgccccaccccgcctttctgctgatcccccagagcgtgaaagagtccgagggcgacctggtcacaccagccggcaacctgaccctgacctgtaccgccagcggcagcgacatcaacgactaccccatctcttgggtccgccaggctcctggcaagggactggaatggatcggcttcatcaacagcggcggcagcacttggtacgccagctgggtcaaaggccggttcaccatcagccggaccagcaccaccgtggacctgaagatgacaagcctgaccaccgacgacaccgccacctacttttgcgccagaggctacagcacctactacggcgacttcaacatctggggccctggcaccctggtcacaatctctagcggcggaggcggcagcggaggtggaggaagtggcggcggaggatccgagctggtcatgacccagacccccagcagcacatctggcgccgtgggcggcaccgtgaccatcaattgccaggccagccagagcatcgacagcaacctggcctggttccagcagaagcccggccagccccccaccctgctgatctacagagcctccaacctggccagcggcgtgccaagcagattcagcggcagcagatctggcaccgagtacaccctgaccatctccggcgtgcagagagaggacgccgctacctattactgcctgggcggcgtgggcaacgtgtcctacagaaccagcttcggcggaggtactgaggtggtcgtcaaatacggaccgccctgccccccttgccctggccagcctcgcgagccccaggtgtacaccctgcctccctcccaggaagagatgaccaagaaccaggtgtccctgacctgcctggtgaagggcttctaccccagcgacatcgccgtggagtgggagagcaacggccagcctgagaacaactacaagaccacccctcccgtgctggacagcgacggcagcttcttcctgtacagccggctgaccgtggacaagagccggtggcaggaaggcaacgtctttagctgcagcgtgatgcacgaggccctgcacaaccactacacccagaagagcctgagcctgtccctgggcaagatgttctgggtgctggtggtggtgggcggggtgctggcctgctacagcctgctggtgacagtggccttcatcatcttttgggtgaaacggggcagaaagaaactcctgtatatattcaaacaaccatttatgagaccagtacaaactactcaagaggaagatggctgtagctgccgatttccagaagaagaagaaggaggatgtgaactgcgggtgaagttcagcagaagcgccgacgcccctgcctaccagcagggccagaatcagctgtacaacgagctgaacctgggcagaagggaagagtacgacgtcctggataagcggagaggccgggaccctgagatgggcggcaagcctcggcggaagaacccccaggaaggcctgtataacgaactgcagaaagacaagatggccgaggcctacagcgagatcggcatgaagggcgagcggaggcggggcaagggccacgacggcctgtatcagggcctgtccaccgccaccaaggatacctacgacgccctgcacatgcaggccctgcccccaaggctcgagggcggcggagagggcagaggaagtcttctaacatgcggtgacgtggaggagaatcccggccctaggatgcttctcctggtgacaagccttctgctctgtgagttaccacacccagcattcctcctgatcccacgcaaagtgtgtaacggaataggtattggtgaatttaaagactcactctccataaatgctacgaatattaaacacttcaaaaactgcacctccatcagtggcgatctccacatcctgccggtggcatttaggggtgactccttcacacatactcctcctctggatccacaggaactggatattctgaaaaccgtaaaggaaatcacagggtttttgctgattcaggcttggcctgaaaacaggacggacctccatgcctttgagaacctagaaatcatacgcggcaggaccaagcaacatggtcagttttctcttgcagtcgtcagcctgaacataacatccttgggattacgctccctcaaggagataagtgatggagatgtgataatttcaggaaacaaaaatttgtgctatgcaaatacaataaactggaaaaaactgtttgggacctccggtcagaaaaccaaaattataagcaacagaggtgaaaacagctgcaaggccacaggccaggtctgccatgccttgtgctcccccgagggctgctggggcccggagcccagggactgcgtctcttgccggaatgtcagccgaggcagggaatgcgtggacaagtgcaaccttctggagggtgagccaagggagtttgtggagaactctgagtgcatacagtgccacccagagtgcctgcctcaggccatgaacatcacctgcacaggacggggaccagacaactgtatccagtgtgcccactacattgacggcccccactgcgtcaagacctgcccggcaggagtcatgggagaaaacaacaccctggtctggaagtacgcagacgccggccatgtgtgccacctgtgccatccaaactgcacctacggatgcactgggccaggtcttgaaggctgtccaacgaatgggcctaagatcccgtccatcgccactgggatggtgggggccctcctcttgctgctggtggtggccctggggatcggcctcttcatgtgagcggccgctctagacccgggctgcaggaattcgatatcaagcttatcgataatcaacctctggattacaaaatttgtgaaagattgactggtattcttaactatgttgctccttttacgctatgtggatacgctgctttaatgcctttgtatcatgctattgcttcccgtatggctttcattttctcctccttgtataaatcctggttgctgtctctttatgaggagttgtggcccgttgtcaggcaacgtggcgtggtgtgcactgtgtttgctgacgcaacccccactggttggggcattgccaccacctgtcagctcctttccgggactttcgctttccccctccctattgccacggcggaactcatcgccgcctgccttgcccgctgctggacaggggctcggctgttgggcactgacaattccgtggtgttgtcggggaaatcatcgtcctttccttggctgctcgcctgtgttgccacctggattctgcgcgggacgtccttctgctacgtcccttcggccctcaatccagcggaccttccttcccgcggcctgctgccggctctgcggcctcttccgcgtcttcgccttcgccctcagacgagtcggatctccctttgggccgcctccccgcatcgataccgtcgactagccgtacctttaagaccaatgacttacaaggcagctgtagatcttagccactttttaaaagaaaaggggggactggaagggctaattcactcccaaagaagacaagatctgctttttgcctgtactgggtctctctggttagaccagatctgagcctgggagctctctggctaactagggaacccactgcttaagcctcaataaagcttgccttgagtgcttcaagtagtgtgtgcccgtctgttgtgtgactctggtaactagagatccctcagacccttttagtcagtgtggaaaatctctagcagaattcgatatcaagcttatcgataccgtcgacctcgagggggggcccggtacccaattcgccctatagtgagtcgtattacaattcactggccgtcgttttacaacgtcgtgactgggaaaaccctggcgttacccaacttaatcgccttgcagcacatccccctttcgccagctggcgtaatagcgaagaggcccgcaccgatcgcccttcccaacagttgcgcagcctgaatggcgaatggaaattgtaagcgttaatattttgttaaaattcgcgttaaatttttgttaaatcagctcattttttaaccaataggccgaaatcggcaaaatcccttataaatcaaaagaatagaccgagatagggttgagtgttgttccagtttggaacaagagtccactattaaagaacgtggactccaacgtcaaagggcgaaaaaccgtctatcagggcgatggcccactacgtgaaccatcaccctaatcaagttttttggggtcgaggtgccgtaaagcactaaatcggaaccctaaagggagcccccgatttagagcttgacggggaaagccggcgaacgtggcgagaaaggaagggaagaaagcgaaaggagcgggcgctagggcgctggcaagtgtagcggtcacgctgcgcgtaaccaccacacccgccgcgcttaatgcgccgctacagggcgcgtcaggtggcacttttcggggaaatgtgcgcggaacccctatttgtttatttttctaaatacattcaaatatgtatccgctcatgagacaataaccctgataaatgcttcaataatattgaaaaaggaagagtatgagtattcaacatttccgtgtcgcccttattcccttttttgcggcattttgccttcctgtttttgctcacccagaaacgctggtgaaagtaaaagatgctgaagatcagttgggtgcacgagtgggttacatcgaactggatctcaacagcggtaagatccttgagagttttcgccccgaagaacgttttccaatgatgagcacttttaaagttctgctatgtggcgcggtattatcccgtattgacgccgggcaagagcaactcggtcgccgcatacactattctcagaatgacttggttgagtactcaccagtcacagaaaagcatcttacggatggcatgacagtaagagaattatgcagtgctgccataaccatgagtgataacactgcggccaacttacttctgacaacgatcggaggaccgaaggagctaaccgcttttttgcacaacatgggggatcatgtaactcgccttgatcgttgggaaccggagctgaatgaagccataccaaacgacgagcgtgacaccacgatgcctgtagcaatggcaacaacgttgcgcaaactattaactggcgaactacttactctagcttcccggcaacaattaatagactggatggaggcggataaagttgcaggaccacttctgcgctcggcccttccggctggctggtttattgctgataaatctggagccggtgagcgtgggtctcgcggtatcattgcagcactggggccagatggtaagccctcccgtatcgtagttatctacacgacggggagtcaggcaactatggatgaacgaaatagacagatcgctgagataggtgcctcactgattaagcattggtaactgtcagaccaagtttactcatatatactttagattgatttaaaacttcatttttaatttaaaaggatctaggtgaagatcctttttgataatctcatgaccaaaatcccttaacgtgagttttcgttccactgagcgtcagaccccgtagaaaagatcaaaggatcttcttgagatcctttttttctgcgcgtaatctgctgcttgcaaacaaaaaaaccaccgctaccagcggtggtttgtttgccggatcaagagctaccaactctttttccgaaggtaactggcttcagcagagcgcagataccaaatactgttcttctagtgtagccgtagttaggccaccacttcaagaactctgtagcaccgcctacatacctcgctctgctaatcctgttaccagtggctgctgccagtggcgataagtcgtgtcttaccgggttggactcaagacgatagttaccggataaggcgcagcggtcgggctgaacggggggttcgtgcacacagcccagcttggagcgaacgacctacaccgaactgagatacctacagcgtgagctatgagaaagcgccacgcttcccgaagggagaaaggcggacaggtatccggtaagcggcagggtcggaacaggagagcgcacgagggagcttccagggggaaacgcctggtatctttatagtcctgtcgggtttcgccacctctgacttgagcgtcgatttttgtgatgctcgtcaggggggcggagcctatggaaaaacgccagcaacgcggcctttttacggttcctggccttttgctggccttttgctcacatgttctttcctgcgttatcccctgattctgtggataaccgtattaccgcctttgagtgagctgataccgctcgccgcagccgaacgaccgagcgcagcgagtcagtgagcgaggaagcggaagagcgcccaatacgcaaaccgcctctccccgcgcgttggccgattcattaatgcagctggcacgacaggtttcccgactggaaagcgggcagtgagcgcaacgcaattaatgtgagttagctcactcattaggcaccccaggctttacactttatgcttccggctcgtatgttgtgtggaattgtgagcggataacaatttcacacaggaaacagctatgaccatgattacgccaagctcgaaattaaccctcactaaagggaacaaaagctggagctccaccgcggtggcggcctcgaggtcgagatccggtcgaccagcaaccatagtcccgcccctaactccgcccatcccgcccctaactccgcccagttccgcccattctccgccccatggctgactaattttttttatttatgcagaggccgaggccgcctcggcctctgagctattccagaagtagtgaggaggcttttttggaggcctaggcttttgcaaaaagcttcgacggtatcgattggctcatgtccaacattaccgccatgttgacattgattattgactagttattaatagtaatcaattacggggtcattagttcatagcccatatatggagttccgcgttacataacttacggtaaatggcccgcctggctgaccgcccaacgacccccgcccattgacgtcaataatgacgtatgttcccatagtaacgccaatagggactttccattgacgtcaatgggtggagtatttacggtaaactgcccacttggcagtacatcaagtgtatcatatgccaagtacgccccctattgacgtcaatgacggtaaatggcccgcctggcattatgcccagtacatgaccttatgggactttcctacttggcagtacatctacgtattagtcatcgctattaccatggtgatgcggttttggcagtacatcaatgggcgtggatagcggtttgactcacggggatttccaagtctccaccccattgacgtcaatgggagtttgttttggcaccaaaatcaacgggactttccaaaatgtcgtaacaactccgccccattgacgcaaatgggcggtaggcgtgtacggaattcggagtggcgagccctcagatcctgcatataagcagctgctttttgcctgtactgggtctctctg

SEQ ID NO: 48 - protein, 838 aa, synthetic construct
  REGION 1..838: note = Synthetic
MLLLVTSLLLCELPHPAFLLIPQSVKESEGDLVTPAGNLTLTCTASGSDINDYPISWVRQAPGKGLEWIGFINSGGSTWYASWVKGRFTISRTSTTVDLKMTSLTTDDTATYFCARGYSTYYGDFNIWGPGTLVTISSGGGGSGGGGSGGGGSELVMTQTPSSTSGAVGGTVTINCQASQSIDSNLAWFQQKPGQPPTLLIYRASNLASGVPSRFSGSRSGTEYTLTISGVQREDAATYYCLGGVGNVSYRTSFGGGTEVVVKESKYGPPCPPCPMFWVLVVVGGVLACYSLLVTVAFIIFWVKRGRKKLLYIFKQPFMRPVQTTQEEDGCSCRFPEEEEGGCELRVKFSRSADAPAYQQGQNQLYNELNLGRREEYDVLDKRRGRDPEMGGKPRRKNPQEGLYNELQKDKMAEAYSEIGMKGERRRGKGHDGLYQGLSTATKDTYDALHMQALPPRLEGGGEGRGSLLTCGDVEENPGPRMLLLVTSLLLCELPHPAFLLIPRKVCNGIGIGEFKDSLSINATNIKHFKNCTSISGDLHILPVAFRGDSFTHTPPLDPQELDILKTVKEITGFLLIQAWPENRTDLHAFENLEIIRGRTKQHGQFSLAVVSLNITSLGLRSLKEISDGDVIISGNKNLCYANTINWKKLFGTSGQKTKIISNRGENSCKATGQVCHALCSPEGCWGPEPRDCVSCRNVSRGRECVDKCNLLEGEPREFVENSECIQCHPECLPQAMNITCTGRGPDNCIQCAHYIDGPHCVKTCPAGVMGENNTLVWKYADAGHVCHLCHPNCTYGCTGPGLEGCPTNGPKIPSIATGMVGALLLLLVVALGIGLFM

SEQ ID NO: 49 - protein, 119 aa, synthetic construct
  REGION 1..119: note = Synthetic
ESKYGPPCPPCPGQPREPQVYTLPPSQEEMTKNQVSLTCLVKGFYPSDIAVEWESNGQPENNYKTTPPVLDSDGSFFLYSRLTVDKSRWQEGNVFSCSVMHEALHNHYTQKSLSLSLGK

SEQ ID NO: 50 - protein, 229 aa, synthetic construct
  REGION 1..229: note = Synthetic
ESKYGPPCPPCPAPEFLGGPSVFLFPPKPKDTLMISRTPEVTCVVVDVSQEDPEVQFNWYVDGVEVHNAKTKPREEQFNSTYRVVSVLTVLHQDWLNGKEYKCKVSNKGLPSSIEKTISKAKGQPREPQVYTLPPSQEEMTKNQVSLTCLVKGFYPSDIAVEWESNGQPENNYKTTPPVLDSDGSFFLYSRLTVDKSRWQEGNVFSCSVMHEALHNHYTQKSLSLSLGK

SEQ ID NO: 51 - protein, 9 aa, synthetic construct
  REGION 1..9: note = Synthetic
YGPPCPPCP

SEQ ID NO: 52 - protein, 10 aa, synthetic construct
  REGION 1..10: note = Synthetic
KYGPPCPPCP

SEQ ID NO: 53 - protein, 14 aa, synthetic construct
  REGION 1..14: note = Synthetic
EVVVKYGPPCPPCP

SEQ ID NO: 54 - DNA, 2529 bp, synthetic construct
  misc_feature 1..2529: note = Synthetic
  source 1..2529: mol_type = other DNA
atgcttctcctggtgacaagccttctgctctgtgagttaccacacccagcattcctcctgatcccagatatccagatgacccagtccccgagctccctgtccgcctctgtgggcgatagggtcaccatcacctgccgtgccagtcaggatgtgaatactgctgtagcctggtatcaacagaaaccaggaaaagctccgaaactactgatttactcggcatccttcctctactctggagtcccttctcgcttctctggttccagatctgggacggatttcactctgaccatcagcagtctgcagccggaagacttcgcaacttattactgtcagcaacattatactactcctcccacgttcggacagggtaccaaggtggagatcaaaggcagtactagcggcggtggctccgggggcggatccggtgggggcggcagcagcgaggttcagctggtggagtctggcggtggcctggtgcagccagggggctcactccgtttgtcctgtgcagcttctggcttcaacattaaagacacctatatacactgggtgcgtcaggccccgggtaagggcctggaatgggttgcaaggatttatcctacgaatggttatactagatatgccgatagcgtcaagggccgtttcactataagcgcagacacatccaaaaacacagcctacctgcagatgaacagcctgcgtgctgaggacactgccgtctattattgttctagatggggaggggacggcttctatgctatggactactggggtcaaggaaccctggtcaccgtctcgagtgagagcaagtacggaccgccctgccccccttgccctatgttctgggtgctggtggtggtcggaggcgtgctggcctgctacagcctgctggtcaccgtggccttcatcatcttttgggtgaaacggggcagaaagaaactcctgtatatattcaaacaaccatttatgagaccagtacaaactactcaagaggaagatggctgtagctgccgatttccagaagaagaagaaggaggatgtgaactgcgggtgaagttcagcagaagcgccgacgcccctgcctaccagcagggccagaatcagctgtacaacgagctgaacctgggcagaagggaagagtacgacgtcctggataagcggagaggccgggaccctgagatgggcggcaagcctcggcggaagaacccccaggaaggcctgtataacgaactgcagaaagacaagatggccgaggcctacagcgagatcggcatgaagggcgagcggaggcggggcaagggccacgacggcctgtatcagggcctgtccaccgccaccaaggatacctacgacgccctgcacatgcaggccctgcccccaaggctcgagggcggcggagagggcagaggaagtcttctaacatgcggtgacgtggaggagaatcccggccctaggatgcttctcctggtgacaagccttctgctctgtgagttaccacacccagcattcctcctgatcccacgcaaagtgtgtaacggaataggtattggtgaatttaaagactcactctccataaatgctacgaatattaaacacttcaaaaactgcacctccatcagtggcgatctccacatcctgccggtggcatttaggggtgactccttcacacatactcctcctctggatccacaggaactggatattctgaaaaccgtaaaggaaatcacagggtttttgctgattcaggcttggcctgaaaacaggacggacctccatgcctttgagaacctagaaatcatacgcggcaggaccaagcaacatggtcagttttctcttgcagtcgtcagcctgaacataacatccttgggattacgctccctcaaggagataagtgatggagatgtgataatttcaggaaacaaaaatttgtgctatgcaaatacaataaactggaaaaaactgtttgggacctccggtcagaaaaccaaaattataagcaacagaggtgaaaacagctgcaaggccacaggccaggtctgccatgccttgtgctcccccgagggctgctggggcccggagcccagggactgcgtctcttgccggaatgtcagccgaggcagggaatgcgtggacaagtgcaaccttctggagggtgagccaagggagtttgtggagaactctgagtgcatacagtgccacccagagtgcctgcctcaggccatgaacatcacctgcacaggacggggaccagacaactgtatccagtgtgcccactacattgacggcccccactgcgtcaagacctgcccggcaggagtcatgggagaaaacaacaccctggtctggaagtacgcagacgccggccatgtgtgccacctgtgccatccaaactgcacctacggatgcactgggccaggtcttgaaggctgtccaacgaatgggcctaagatcccgtccatcgccactgggatggtgggggccctcctcttgctgctggtggtggccctggggatcggcctcttcatgtga

SEQ ID NO: 55 - DNA, 2850 bp, synthetic construct
  misc_feature 1..2850: note = Synthetic
  source 1..2850: mol_type = other DNA
atgcttctcctggtgacaagccttctgctctgtgagttaccacacccagcattcctcctgatcccagatatccagatgacccagtccccgagctccctgtccgcctctgtgggcgatagggtcaccatcacctgccgtgccagtcaggatgtgaatactgctgtagcctggtatcaacagaaaccaggaaaagctccgaaactactgatttactcggcatccttcctctactctggagtcccttctcgcttctctggttccagatctgggacggatttcactctgaccatcagcagtctgcagccggaagacttcgcaacttattactgtcagcaacattatactactcctcccacgttcggacagggtaccaaggtggagatcaaaggcagtactagcggcggtggctccgggggcggatccggtgggggcggcagcagcgaggttcagctggtggagtctggcggtggcctggtgcagccagggggctcactccgtttgtcctgtgcagcttctggcttcaacattaaagacacctatatacactgggtgcgtcaggccccgggtaagggcctggaatgggttgcaaggatttatcctacgaatggttatactagatatgccgatagcgtcaagggccgtttcactataagcgcagacacatccaaaaacacagcctacctgcagatgaacagcctgcgtgctgaggacactgccgtctattattgttctagatggggaggggacggcttctatgctatggactactggggtcaaggaaccctggtcaccgtctcgagtgagagcaagtacggaccgccctgccccccttgccctggccagcctagagaaccccaggtgtacaccctgcctcccagccaggaagagatgaccaagaaccaggtgtccctgacctgcctggtcaaaggcttctaccccagcgatatcgccgtggaatgggagagcaacggccagcccgagaacaactacaagaccaccccccctgtgctggacagcgacggcagcttcttcctgtactcccggctgaccgtggacaagagccggtggcaggaaggcaacgtcttcagctgcagcgtgatgcacgaggccctgcacaaccactacacccagaagtccctgagcctgagcctgggcaagatgttctgggtgctggtggtggtcggaggcgtgctggcctgctacagcctgctggtcaccgtggccttcatcatcttttgggtgaaacggggcagaaagaaactcctgtatatattcaaacaaccatttatgagaccagtacaaactactcaagaggaagatggctgtagctgccgatttccagaagaagaagaaggaggatgtgaactgcgggtgaagttcagcagaagcgccgacgcccctgcctaccagcagggccagaatcagctgtacaacgagctgaacctgggcagaagggaagagtacgacgtcctggataagcggagaggccgggaccctgagatgggcggcaagcctcggcggaagaacccccaggaaggcctgtataacgaactgcagaaagacaagatggccgaggcctacagcgagatcggcatgaagggcgagcggaggcggggcaagggccacgacggcctgtatcagggcctgtccaccgccaccaaggatacctacgacgccctgcacatgcaggccctgcccccaaggctcgagggcggcggagagggcagaggaagtcttctaacatgcggtgacgtggaggagaatcccggccctaggatgcttctcctggtgacaagccttctgctctgtgagttaccacacccagcattcctcctgatcccacgcaaagtgtgtaacggaataggtattggtgaatttaaagactcactctccataaatgctacgaatattaaacacttcaaaaactgcacctccatcagtggcgatctccacatcctgccggtggcatttaggggtgactccttcacacatactcctcctctggatccacaggaactggatattctgaaaaccgtaaaggaaatcacagggtttttgctgattcaggcttggcctgaaaacaggacggacctccatgcctttgagaacctagaaatcatacgcggcaggaccaagcaacatggtcagttttctcttgcagtcgtcagcctgaacataacatccttgggattacgctccctcaaggagataagtgatggagatgtgataatttcaggaaacaaaaatttgtgctatgcaaatacaataaactggaaaaaactgtttgggacctccggtcagaaaaccaaaattataagcaacagaggtgaaaacagctgcaaggccacaggccaggtctgccatgccttgtgctcccccgagggctgctggggcccggagcccagggactgcgtctcttgccggaatgtcagccgaggcagggaatgcgtggacaagtgcaaccttctggagggtgagccaagggagtttgtggagaactctgagtgcatacagtgccacccagagtgcctgcctcaggccatgaacatcacctgcacaggacggggaccagacaactgtatccagtgtgcccactacattgacggcccccactgcgtcaagacctgcccggcaggagtcatgggagaaaacaacaccctggtctggaagtacgcagacgccggccatgtgtgccacctgtgccatccaaactgcacctacggatgcactgggccaggtcttgaaggctgtccaacgaatgggcctaagatcccgtccatcgccactgggatggtgggggccctcctcttgctgctggtggtggccctggggatcggcctcttcatgtga

SEQ ID NO: 56 - DNA, 3180 bp, synthetic construct
  misc_feature 1..3180: note = Synthetic
  source 1..3180: mol_type = other DNA
atgcttctcctggtgacaagccttctgctctgtgagttaccacacccagcattcctcctgatcccagatatccagatgacccagtccccgagctccctgtccgcctctgtgggcgatagggtcaccatcacctgccgtgccagtcaggatgtgaatactgctgtagcctggtatcaacagaaaccaggaaaagctccgaaactactgatttactcggcatccttcctctactctggagtcccttctcgcttctctggttccagatctgggacggatttcactctgaccatcagcagtctgcagccggaagacttcgcaacttattactgtcagcaacattatactactcctcccacgttcggacagggtaccaaggtggagatcaaaggcagtactagcggcggtggctccgggggcggatccggtgggggcggcagcagcgaggttcagctggtggagtctggcggtggcctggtgcagccagggggctcactccgtttgtcctgtgcagcttctggcttcaacattaaagacacctatatacactgggtgcgtcaggccccgggtaagggcctggaatgggttgcaaggatttatcctacgaatggttatactagatatgccgatagcgtcaagggccgtttcactataagcgcagacacatccaaaaacacagcctacctgcagatgaacagcctgcgtgctgaggacactgccgtctattattgttctagatggggaggggacggcttctatgctatggactactggggtcaaggaaccctggtcaccgtctcgagtgagagcaagtacggaccgccctgccccccttgccctgcccccgagttcctgggcggacccagcgtgttcctgttcccccccaagcccaaggacaccctgatgatcagccggacccccgaggtgacctgcgtggtggtggacgtgagccaggaagatcccgaggtccagttcaattggtacgtggacggcgtggaagtgcacaacgccaagaccaagcccagagaggaacagttcaacagcacctaccgggtggtgtctgtgctgaccgtgctgcaccaggactggctgaacggcaaagaatacaagtgcaaggtgtccaacaagggcctgcccagcagcatcgaaaagaccatcagcaaggccaagggccagcctcgcgagccccaggtgtacaccctgcctccctcccaggaagagatgaccaagaaccaggtgtccctgacctgcctggtgaagggcttctaccccagcgacatcgccgtggagtgggagagcaacggccagcctgagaacaactacaagaccacccctcccgtgctggacagcgacggcagcttcttcctgtacagccggctgaccgtggacaagagccggtggcaggaaggcaacgtctttagctgcagcgtgatgcacgaggccctgcacaaccactacacccagaagagcctgagcctgtccctgggcaagatgttctgggtgctggtggtggtgggcggggtgctggcctgctacagcctgctggtgacagtggccttcatcatcttttgggtgaaacggggcagaaagaaactcctgtatatattcaaacaaccatttatgagaccagtacaaactactcaagaggaagatggctgtagctgccgatttccagaagaagaagaaggaggatgtgaactgcgggtgaagttcagcagaagcgccgacgcccctgcctaccagcagggccagaatcagctgtacaacgagctgaacctgggcagaagggaagagtacgacgtcctggataagcggagaggccgggaccctgagatgggcggcaagcctcggcggaagaacccccaggaaggcctgtataacgaactgcagaaagacaagatggccgaggcctacagcgagatcggcatgaagggcgagcggaggcggggcaagggccacgacggcctgtatcagggcctgtccaccgccaccaaggatacctacgacgccctgcacatgcaggccctgcccccaaggctcgagggcggcggagagggcagaggaagtcttctaacatgcggtgacgtggaggagaatcccggccctaggatgcttctcctggtgacaagccttctgctctgtgagttaccacacccagcattcctcctgatcccacgcaaagtgtgtaacggaataggtattggtgaatttaaagactcactctccataaatgctacgaatattaaacacttcaaaaactgcacctccatcagtggcgatctccacatcctgccggtggcatttaggggtgactccttcacacatactcctcctctggatccacaggaactggatattctgaaaaccgtaaaggaaatcacagggtttttgctgattcaggcttggcctgaaaacaggacggacctccatgcctttgagaacctagaaatcatacgcggcaggaccaagcaacatggtcagttttctcttgcagtcgtcagcctgaacataacatccttgggattacgctccctcaaggagataagtgatggagatgtgataatttcaggaaacaaaaatttgtgctatgcaaatacaataaactggaaaaaactgtttgggacctccggtcagaaaaccaaaattataagcaacagaggtgaaaacagctgcaaggccacaggccaggtctgccatgccttgtgctcccccgagggctgctggggcccggagcccagggactgcgtctcttgccggaatgtcagccgaggcagggaatgcgtggacaagtgcaaccttctggagggtgagccaagggagtttgtggagaactctgagtgcatacagtgccacccagagtgcctgcctcaggccatgaacatcacctgcacaggacggggaccagacaactgtatccagtgtgcccactacattgacggcccccactgcgtcaagacctgcccggcaggagtcatgggagaaaacaacaccctggtctggaagtacgcagacgccggccatgtgtgccacctgtgccatccaaactgcacctacggatgcactgggccaggtcttgaaggctgtccaacgaatgggcctaagatcccgtccatcgccactgggatggtgggggccctcctcttgctgctggtggtggccctggggatcggcctcttcatgtga